European Patent Specification EP 3 482 769 B1, published May 29, 2024. Title: Covalent Diabodies And Uses Thereof. Applicant: MacroGenics, Inc. The sequence listing filed with the application follows.

SEQUENCE LISTING (322 sequences)

SEQ ID NO: 1 - protein, 13 aa, homo sapiens
EPKSCDKTHTCPP

SEQ ID NO: 2 - protein, 10 aa, homo sapiens
ERKCCVECPP

SEQ ID NO: 3 - protein, 60 aa, homo sapiens
ELKTPLGDTTHTCPRCPEPKSCDTPPPCPRCPEPKSCDTPPPCPRCPEPKSCDTPPPCPR

SEQ ID NO: 4 - protein, 10 aa, homo sapiens
ESKYGPPCPS

SEQ ID NO: 5 - protein, 217 aa, homo sapiens
APELLGGPSVFLFPPKPKDTLMISRTPEVTCVVVDVSHEDPEVKFNWYVDGVEVHNAKTKPREEQYNSTYRVVSVLTVLHQDWLNGKEYKCKVSNKALPAPIEKTISKAKGQPREPQVYTLPPSRDELTKNQVSLTCLVKGFYPSDIAVEWESNGQPENNYKTTPPVLDSDGSFFLYSKLTVDKSRWQQGNVFSCSVMHEALHNHYTQKSLSLSPGK

SEQ ID NO: 6 - protein, 216 aa, homo sapiens
APPVAGPSVFLFPPKPKDTLMISRTPEVTCVVVDVSHEDPEVQFNWYVDGVEVHNAKTKPREEQFNSTFRVVSVLTVVHQDWLNGKEYKCKVSNKGLPAPIEKTISKTKGQPREPQVYTLPPSREEMTKNQVSLTCLVKGFYPSDIAVEWESNGQPENNYKTTPPMLDSDGSFFLYSKLTVDKSRWQQGNVFSCSVMHEALHNHYTQKSLSLSPGK

SEQ ID NO: 7 - protein, 217 aa, homo sapiens
APELLGGPSVFLFPPKPKDTLMISRTPEVTCVVVDVSHEDPEVQFKWYVDGVQVHNAKTKPREQQFNSTFRVVSVLTVLHQNWLDGKEYKCKVSNKALPAPIEKTISKTKGQPREPQVYTLPPSREEMTKNQVSLTCLVKGFYPSDIAVEWESSGQPENNYNTTPPMLDSDGSFFLYSKLTVDKSRWQQGNIFSCSVMHEALHNRFTQKSLSLSPGK

SEQ ID NO: 8 - protein, 217 aa, homo sapiens
APEFLGGPSVFLFPPKPKDTLMISRTPEVTCVVVDVSQEDPEVQFNWYVDGVEVHNAKTKPREEQFNSTYRVVSVLTVLHQDWLNGKEYKCKVSNKGLPSSIEKTISKAKGQPREPQVYTLPPSQEEMTKNQVSLTCLVKGFYPSDIAVEWESNGQPENNYKTTPPVLDSDGSFFLYSRLTVDKSRWQEGNVFSCSVMHEALHNHYTQKSLSLSLGK

SEQ ID NO: 9 - protein, 237 aa, homo sapiens
EIVLTQSPDFQSVTPKEKVTFTCRTSQSIGTNIHWYQQKPDQSPKLLIKEVSESISGVPSRFSGSGSGTDFTLTINSLEAEDAATYYCQQSNTWPFTFGGGTKVEIKGGGSGGGGQVTLRESGPALVKPTQTLTLTCTFSGFSLSTSGMGVGWIRQPPGKALEWLAHIWWDDDKRYNPALKSRLTISKDTSKNQVVLTMTNMDPVDTATYYCAQINPAWFAYWGQGTLVTVSSLGGC

SEQ ID NO: 10 - protein, 8 aa, homo sapiens
GGGSGGGG

SEQ ID NO: 11 - protein, 244 aa, homo sapiens
DIVMTQSPDSLAVSLGERATINCKASQSVDFDGDSFMNWYQQKPGQPPKLLIYTTSNLESGVPDRFSGSGSGTDFTLTISSLQAEDVAVYYCQQSNEDPYTFGQGTKLEIKGGGSGGGGQVQLVQSGAEVKKPGASVKVSCKASGYTFTNYWIHWVRQAPGQGLEWIGVIDPSDTYPNYNKKFKGRVTMTVVVSTSTAYMELRSLRSDDTAVYYCARNGDSDYYSGMDYWGQGTTVTVSSLGGC

SEQ ID NO: 12 - protein, 240 aa, homo sapiens
EIVLTQSPDFQSVTPKEKVTFTCRTSQSIGTNIHWYQQKPDQSPKLLIKEVSESISGVPSRFSGSGSGTDFTLTINSLEAEDAATYYCQQSNTWPFTFGGGTKVEIKGGGSGGGGQVQLVQSGAEVKKPGASVKVSCKASGYTFTNYWIHWVRQAPGQGLEWIGVIDPSDTYPNYNKKFKGRVTMTVVVSTSTAYMELRSLRSDDTAVYYCARNGDSDYYSGMDYWGQGTTVTVSSLGGC

SEQ ID NO: 13 - protein, 241 aa, homo sapiens
DIVMTQSPDSLAVSLGERATINCKASQSVDFDGDSFMNWYQQKPGQPPKLLIYTTSNLESGVPDRFSGSGSGTDFTLTISSLQAEDVAVYYCQQSNEDPYTFGQGTKLEIKGGGSGGGGQVTLRESGPALVKPTQTLTLTCTFSGFSLSTSGMGVGWIRQPPGKALEWLAHIWWDDDKRYNPALKSRLTISKDTSKNQVVLTMTNMDPVDTATYYCAQINPAWFAYWGQGTLVTVSSLGGC

SEQ ID NO: 14 - protein, 470 aa, homo sapiens
EIVLTQSPDFQSVTPKEKVTFTCRTSQSIGTNIHWYQQKPDQSPKLLIKEVSESISGVPSRFSGSGSGTDFTLTINSLEAEDAATYYCQQSNTWPFTFGGGTKVEIKGGGSGGGGQVTLRESGPALVKPTQTLTLTCTFSGFSLSTSGMGVGWIRQPPGKALEWLAHIWWDDDKRYNPALKSRLTISKDTSKNQVVLTMTNMDPVDTATYYCAQINPAWFAYWGQGTLVTVSSLGGCVEPKSCDKTHTCPPCPAPELLGGPSVFLFPPKPKDTLMISRTPEVTCVVVDVSHEDPEVKFNWYVDGVEVHNAKTKPREEQYNSTYRVVSVLTVLHQDWLNGKEYKCKVSNKALPAPIEKTISKAKGQPREPQVYTLPPSRDELTKNQVSLTCLVKGFYPSDIAVEWESNGQPENNYKTTPPVLDSDGSFFLYSKLTVDKSRWQQGNVFSCSVMHEALHNHYTQKSLSLSPGK

SEQ ID NO: 15 - protein, 477 aa, homo sapiens
DIVMTQSPDSLAVSLGERATINCKASQSVDFDGDSFMNWYQQKPGQPPKLLIYTTSNLESGVPDRFSGSGSGTDFTLTISSLQAEDVAVYYCQQSNEDPYTFGQGTKLEIKGGGSGGGGQVQLVQSGAEVKKPGASVKVSCKASGYTFTNYWIHWVRQAPGQGLEWIGVIDPSDTYPNYNKKFKGRVTMTVVVSTSTAYMELRSLRSDDTAVYYCARNGDSDYYSGMDYWGQGTTVTVSSLGGCVEPKSCDKTHTCPPCPAPELLGGPSVFLFPPKPKDTLMISRTPEVTCVVVDVSHEDPEVKFNWYVDGVEVHNAKTKPREEQYNSTYRVVSVLTVLHQDWLNGKEYKCKVSNKALPAPIEKTISKAKGQPREPQVYTLPPSRDELTKNQVSLTCLVKGFYPSDIAVEWESNGQPENNYKTTPPVLDSDGSFFLYSKLTVDKSRWQQGNVFSCSVMHEALHNHYTQKSLSLSPGK

SEQ ID NO: 16 - protein, 243 aa, homo sapiens
EIVLTQSPDFQSVTPKEKVTFTCRTSQSIGTNIHWYQQKPDQSPKLLIKEVSESISGVPSRFSGSGSGTDFTLTINSLEAEDAATYYCQQSNTWPFTFGGGTKVEIKGGGSGGGGQVTLRESGPALVKPTQTLTLTCTFSGFSLSTSGMGVGWIRQPPGKALEWLAHIWWDDDKRYNPALKSRLTISKDTSKNQVVLTMTNMDPVDTATYYCAQINPAWFAYWGQGTLVTVSSLGGCFNRGEC

SEQ ID NO: 17 - protein, 10 aa, artificial
  linker plus C-terminus of human IgG-kappa chain
LGGCFNRGEC

SEQ ID NO: 18 - protein, 477 aa, homo sapiens
DIVMTQSPDSLAVSLGERATINCKASQSVDFDGDSFMNWYQQKPGQPPKLLIYTTSNLESGVPDRFSGSGSGTDFTLTISSLQAEDVAVYYCQQSNEDPYTFGQGTKLEIKGGGSGGGGQVQLVQSGAEVKKPGASVKVSCKASGYTFTNYWIHWVRQAPGQGLEWIGVIDPSDTYPNYNKKFKGRVTMTVVVSTSTAYMELRSLRSDDTAVYYCARNGDSDYYSGMDYWGQGTTVTVSSLGGCAEPKSCDKTHTCPPCPAPELLGGPSVFLFPPKPKDTLMISRTPEVTCVVVDVSHEDPEVKFNWYVDGVEVHNAKTKPREEQYNSTYRVVSVLTVLHQDWLNGKEYKCKVSNKALPAPIEKTISKAKGQPREPQVYTLPPSRDELTKNQVSLTCLVKGFYPSDIAVEWESNGQPENNYKTTPPVLDSDGSFFLYSKLTVDKSRWQQGNVFSCSVMHEALHNHYTQKSLSLSPGK

SEQ ID NO: 19 - protein, 485 aa, homo sapiens
VEPKSCDKTHTCPPCPAPELLGGPSVFLFPPKPKDTLMISRTPEVTCVVVDVSHEDPEVKFNWYVDGVEVHNAKTKPREEQYNSTYRVVSVLTVLHQDWLNGKEYKCKVSNKALPAPIEKTISKAKGQPREPQVYTLPPSRDELTKNQVSLTCLVKGFYPSDIAVEWESNGQPENNYKTTPPVLDSDGSFFLYSKLTVDKSRWQQGNVFSCSVMHEALHNHYTQKSLSLSPGKGGGSGGGGDIVMTQSPDSLAVSLGERATINCKASQSVDFDGDSFMNWYQQKPGQPPKLLIYTTSNLESGVPDRFSGSGSGTDFTLTISSLQAEDVAVYYCQQSNEDPYTFGQGTKLEIKGGGSGGGGQVQLVQSGAEVKKPGASVKVSCKASGYTFTNYWIHWVRQAPGQGLEWIGVIDPSDTYPNYNKKFKGRVTMTVVVSTSTAYMELRSLRSDDTAVYYCARNGDSDYYSGMDYWGQGTTVTVSSLGGC

SEQ ID NO: 20 - protein, 469 aa, homo sapiens
APELLGGPSVFLFPPKPKDTLMISRTPEVTCVVVDVSHEDPEVKFNWYVDGVEVHNAKTKPREEQYNSTYRVVSVLTVLHQDWLNGKEYKCKVSNKALPAPIEKTISKAKGQPREPQVYTLPPSRDELTKNQVSLTCLVKGFYPSDIAVEWESNGQPENNYKTTPPVLDSDGSFFLYSKLTVDKSRWQQGNVFSCSVMHEALHNHYTQKSLSLSPGKGGGSGGGGDIVMTQSPDSLAVSLGERATINCKASQSVDFDGDSFMNWYQQKPGQPPKLLIYTTSNLESGVPDRFSGSGSGTDFTLTISSLQAEDVAVYYCQQSNEDPYTFGQGTKLEIKGGGSGGGGQVQLVQSGAEVKKPGASVKVSCKASGYTFTNYWIHWVRQAPGQGLEWIGVIDPSDTYPNYNKKFKGRVTMTVVVSTSTAYMELRSLRSDDTAVYYCARNGDSDYYSGMDYWGQGTTVTVSSLGGC

SEQ ID NO: 21 - protein, 466 aa, homo sapiens
EIVLTQSPDFQSVTPKEKVTFTCRTSQSIGTNIHWYQQKPDQSPKLLIKEVSESISGVPSRFSGSGSGTDFTLTINSLEAEDAATYYCQQSNTWPFTFGCGTKVEIKGGGSGGGGQVTLRESGPALVKPTQTLTLTCTFSGFSLSTSGMGVGWIRQPPGKALEWLAHIWWDDDKRYNPALKSRLTISKDTSKNQVVLTMTNMDPVDTATYYCAQINPAWFAYWGQGTLVTVSSVEPKSCDKTHTCPPCPAPELLGGPSVFLFPPKPKDTLMISRTPEVTCVVVDVSHEDPEVKFNWYVDGVEVHNAKTKPREEQYNSTYRVVSVLTVLHQDWLNGKEYKCKVSNKALPAPIEKTISKAKGQPREPQVYTLPPSRDELTKNQVSLTCLVKGFYPSDIAVEWESNGQPENNYKTTPPVLDSDGSFFLYSKLTVDKSRWQQGNVFSCSVMHEALHNHYTQKSLSLSPGK

SEQ ID NO: 22 - protein, 246 aa, homo sapiens
DIVMTQSPDSLAVSLGERATINCKASQSVDFDGDSFMNWYQQKPGQPPKLLIYTTSNLESGVPDRFSGSGSGTDFTLTISSLQAEDVAVYYCQQSNEDPYTFGQGTKLEIKGGGSGGGGQVQLVQSGAEVKKPGASVKVSCKASGYTFTNYWIHWVRQAPGQCLEWIGVIDPSDTYPNYNKKFKGRVTMTVVVSTSTAYMELRSLRSDDTAVYYCARNGDSDYYSGMDYWGQGTTVTVSSFNRGEC

SEQ ID NO: 23 - protein, 6 aa, homo sapiens
FNRGEC

SEQ ID NO: 24 - protein, 5 aa, artificial
  2B6 heavy chain variable region  CDR1
NYWIH

SEQ ID NO: 25 - protein, 5 aa, artificial
  3H7 Heavy chain variable region CDR1
DAWMD

SEQ ID NO: 26 - protein, 17 aa, artificial
  2B6 Heavy chain variable region  CDR2
VIDPSDTYPNYNKKFKG

SEQ ID NO: 27 - protein, 19 aa, Artificial Sequence
  3H7 Heavy chain variable region CDR2
EIRNKANNLATYYAESVKG

SEQ ID NO: 28 - protein, 12 aa, artificial
  2B6 Heavy chain variable region  CDR3
NGDSDYYSGMDY

SEQ ID NO: 29 - protein, 6 aa, artificial
  3H7 heavy chain variable region  CDR3
YSPFAY

SEQ ID NO: 30 - protein, 11 aa, artificial
  2B6 Light chain variable region  CDR1
RTSQSIGTNIH

SEQ ID NO: 31 - protein, 11 aa, artificial
  3H7 light chain variable region  CDR1
RASQEISGYLS

SEQ ID NO: 32 - protein, 7 aa, artificial
  2B6 light chain variable region  CDR2
NVSESIS

SEQ ID NO: 33 - protein, 7 aa, artificial
  2B6 light chain variable region  CDR2
YVSESIS

SEQ ID NO: 34 - protein, 7 aa, artificial
  2B6 light chain variable region CDR2
YASESIS

SEQ ID NO: 35 - protein, 7 aa, artificial
  3H7 light chain variable region CDR2
AASTLDS

SEQ ID NO: 36 - protein, 9 aa, artificial
  2B6 Light chain variable region CDR3
QQSNTWPFT

SEQ ID NO: 37 - protein, 9 aa, artificial
  3H7 light chain variable region CDR3
LQYVSYPYT

SEQ ID NO: 38 - protein, 121 aa, artificial
  2B6 heavy chain variable region
QVQLVQSGAEVKKPGASVKVSCKASGYTFTNYWIHWVRQAPGQGLEWMGVIDPSDTYPNYNKKFKGRVTMTTDTSTSTAYMELRSLRSDDTAVYYCARNGDSDYYSGMDYWGQGTTVTVSS

SEQ ID NO: 39 - protein, 107 aa, artificial
  2B6 light chain variable region  Hu2B6VL-1
EIVLTQSPDFQSVTPKEKVTITCRTSQSIGTNIHWYQQKPDQSPKLLIKNVSESISGVPSRFSGSGSGTDFTLTINSLEAEDAATYYCQQSNTWPFTFGGGTKVEIK

SEQ ID NO: 40 - protein, 107 aa, artificial
  Humanized 2B6 light chain variable region Hu2B6VL-2
EIVLTQSPDFQSVTPKEKVTITCRTSQSIGTNIHWYQQKPDQSPKLLIKYVSESISGVPSRFSGSGSGTDFTLTINSLEAEDAATYYCQQSNTWPFTFGGGTKVEIK

SEQ ID NO: 41 - protein, 107 aa, artificial
  Humanized 2B6 light chain variable region  Hu2B6VL-3
EIVLTQSPDFQSVTPKEKVTITCRTSQSIGTNIHWYQQKPDQSPKLLIKYASESISGVPSRFSGSGSGTDFTLTINSLEAEDAATYYCQQSNTWPFTFGGGTKVEIK

SEQ ID NO: 42 - protein, 107 aa, Mus sp.
DIQMTQSPSSLSASLGERVSLTCRASQEISGYLSWLQQKPDGTIRRLIYAASTLDSGVPKRFSGSWSGSDYSLTISSLESEDFADYYCLQYVSYPYTFGGGTKLEIK

SEQ ID NO: 43 - protein, 9 aa, artificial
  IgG binding site of FcgammaRIIB receptor
KKFSRSDPN

SEQ ID NO: 44 - protein, 9 aa, artificial
  IgG binding site of FcgammaRIIB receptor
QKFSRLDPN

SEQ ID NO: 45 - protein, 9 aa, artificial
  IgG binding site of FcgammaRIIB receptor
QKFSRLDPT

SEQ ID NO: 46 - protein, 9 aa, artificial
  IgG binding site of FcgammaRIIB receptor
KKFSRLDPT

SEQ ID NO: 47 - protein, 9 aa, artificial
  IgG binding site of FcgammaRIIB receptor
QKFSHLDPT

SEQ ID NO: 48 - protein, 9 aa, artificial
  IgG binding site of FcgammaRIIB receptor
KKFSHLDPT

SEQ ID NO: 49 - protein, 9 aa, artificial
  IgG binding site of FcgammaRIIB receptor
QKFSRLDPN

SEQ ID NO: 50 - protein, 9 aa, artificial
  IgG binding site for FcgammaRIIB receptor
KKFSRSDPN

SEQ ID NO: 51 - protein, 9 aa, artificial
  IgG binding site of FcgammaRIIB receptor
QKFSRLDPT

SEQ ID NO: 52 - protein, 9 aa, artificial
  IgG binding site of FcgammaRIIB receptor
QKFSHLDPT

SEQ ID NO: 53 - protein, 9 aa, artificial
  IgG binding site of FcgammaRIIB receptor
KKFSRLDPT

SEQ ID NO: 54 - protein, 9 aa, artificial
  IgG binding site of FcgammaRIIB receptor
KKFSHLDPT

SEQ ID NO: 55 - DNA, 36 bp, artificial
  Primer  Lgh321F
cgagctagctctagatgagatcacagttctctctac

SEQ ID NO: 56 - DNA, 47 bp, artificial
  Primer  Lgh318R
gcctccgcctccggatccgcctcctttgatctccaccttggtccctc

SEQ ID NO: 57 - DNA, 47 bp, artificial
  Primer Lgh319F
ggaggcggatccggaggcggaggccaggttcagctggtgcagtctgg

SEQ ID NO: 58 - DNA, 43 bp, artificial
  Primer  Lgh320R
tttgaattctagcagcctcccagtgaggagacggtgaccgtgg

SEQ ID NO: 59 - DNA, 46 bp, artificial
  Primer Lgh315R
gcctccgcctccggatccgcctcctttgatctcaagcttggtcccc

SEQ ID NO: 60 - DNA, 48 bp, artificial
  Primer Lgh316F
ggaggcggatccggaggcggaggccaggttaccctgagagagtctggc

SEQ ID NO: 61 - DNA, 47 bp, artificial
  Primer Lgh317R
tttgaattcctagcagcctcccagtgagctcacagtgaccagagtcc

SEQ ID NO: 62 - DNA, 27 bp, artificial
  Primer Lgh339R
ctcaacgcagcctcccagtgagctcac

SEQ ID NO: 63 - DNA, 31 bp, artificial
  Primer Lgh340R
aacgcagcctcccagtgaggagacggtgacc

SEQ ID NO: 64 - DNA, 27 bp, artificial
  Primer Lgh366R
tttgaattctatttacccggagacagg

SEQ ID NO: 65 - DNA, 33 bp, artificial
  Primer Lhg367F
ctgggaggctgcgcagagcccaaatcttgtgac

SEQ ID NO: 66 - DNA, 33 bp, artificial
  Primer Lgh368R
gtcacaagatttgggctctgcgcagcctcccag

SEQ ID NO: 67 - DNA, 50 bp, artificial
  Primer Lgh369R
tttgaattctaacactctcccctgttgaagcagcctcccagtgaggagac

SEQ ID NO: 68 - protein, 118 aa, artificial
  humanized anti-CD16A Heavy Chain Variable Region Hu3G8VH-1
QVTLRESGPALVKPTQTLTLTCTFSGFSLSTSGMGVGWIRQPPGKALEWLAHIWWDDDKRYNPALKSRLTISKDTSKNQVVLTMTNMDPVDTATYYCARINPAWFAYWGQGTLVTVSS

SEQ ID NO: 69 - protein, 118 aa, artificial
  Humanized anti-CD16A heavy chain variable region  Hu3G8VH-5
QVTLRESGPALVKPTQTLTLTCTFSGFSLSTSGMGVGWIRQPPGKALEWLAHIWWDDDKRYNPALKSRLTISKDTSKNQVVLTMTNMDPVDTATYYCAQINPAWFAYWGQGTLVTVSS

SEQ ID NO: 70 - protein, 117 aa, artificial
  Humanized anti-CD16A heavy chain variable region Hu3G8VH-22
QVTLRESGPALVKPTQTLTLTCTFSGFSLSTSGVGVGWIRQPPGKALEWLAHIWWDDDKRYSPSLKSRLTISKDTSKNQVVLTMTNMDPVDTATYYCARINPAYFAYWGQGTLVTVS

SEQ ID NO: 71 - protein, 111 aa, artificial
  Humanized anti-CD16A light chain variable region Hu3G8VL-1
DIVMTQSPDSLAVSLGERATINCKASQSVDFDGDSFMNWYQQKPGQPPKLLIYTTSNLESGVPDRFSGSGSGTDFTLTISSLQAEDVAVYYCQQSNEDPYTFGQGTKLEIK

SEQ ID NO: 72 - protein, 111 aa, artificial
  Humanized anti-CD16A light chain variable region  Hu3G8VL-43
DIVMTQSPDSLAVSLGERATINCKSSQSVDFDGDSFMNWYQQKPGQPPKLLIYTTSSLESGVPDRFSGSGSGTDFTLTISSLQAEDVAVYYCQQSNSDPYTFGQGTKLEIK

SEQ ID NO: 73 - protein, 111 aa, artificial
  Humanized anti-CD16A light chain variable region  Hu3G8VL-22
DIVMTQSPDSLAVSLGERATINCKSSQSVDFDGDSFMNWYQQKPGQPPKLLIYTTSNLETGVPDRFSGSGSGTDFTLTISSLQAEDVAVYYCQQSNSDPYTFGQGTKLEIK

SEQ ID NO: 74 - DNA, 24 bp, DNA sequence of SEQ ID NO:10
ggaggcggatccggaggcggaggc

SEQ ID NO: 75 - DNA, 18 bp, homo sapiens
ttcaacaggggagagtgt

SEQ ID NO: 76 - DNA, 30 bp, artificial
  Linker plus C-terminus of human IgG kappa chain
ctgggaggctgcttcaacaggggagagtgt

SEQ ID NO: 77 - protein, 6 aa, homo sapiens
VEPKSC

SEQ ID NO: 78 - DNA, 18 bp, homo sapiens
gttgagcccaaatcttgt

SEQ ID NO: 79 - protein, 118 aa, homo sapiens
QVTLKESGPGILQPSQTLSLTCSFSGFSLRTSGMGVGWIRQPSGKGLEWLAHIWWDDDKRYNPALKSRLTISKDTSSNQVFLKIASVDTADTATYYCAQINPAWFAYWGQGTLVTVSS

SEQ ID NO: 80 - DNA, 354 bp, homo sapiens
caggttaccctgaaagagtctggccctgggatattgcagccctcccagaccctcagtctgacttgttctttctctgggttttcactgaggacttctggtatgggtgtaggctggattcgtcagccttcagggaagggtctagagtggctggcacacatttggtgggatgatgacaagcgctataatccagccctgaagagccgactgacaatctccaaggatacctccagcaaccaggtattcctcaaaatcgccagtgtggacactgcagatactgccacatactactgtgctcaaataaaccccgcctggtttgcttactggggccaagggactctggtcactgtgagctca

SEQ ID NO: 81 - DNA, 354 bp, homo sapiens
caggttaccctgagagagtctggccctgcgctggtgaagcccacacagaccctcacactgacttgtaccttctctgggttttcactgagcacttctggtatgggtgtaggctggattcgtcagcctcccgggaaggctctagagtggctggcacacatttggtgggatgatgacaagcgctataatccagccctgaagagccgactgacaatctccaaggatacctccaaaaaccaggtagtcctcacaatgaccaacatggaccctgtggatactgccacatactactgtgctcaaataaaccccgcctggtttgcttactggggccaagggactctggtcactgtgagctca

SEQ ID NO: 82 - protein, 111 aa, homo sapiens
DTVLTQSPASLAVSLGQRATISCKASQSVDFDGDSFMNWYQQKPGQPPKLLIYTTSNLESGIPARFSASGSGTDFTLNIHPVEEEDTATYYCQQSNEDPYTFGGGTKLEIK

SEQ ID NO: 83 - DNA, 333 bp, homo sapiens
gacactgtgctgacccaatctccagcttctttggctgtgtctctagggcagagggccaccatctcctgcaaggccagccaaagtgttgattttgatggtgatagttttatgaactggtaccaacagaaaccaggacagccacccaaactcctcatctatactacatccaatctagaatctgggatcccagccaggtttagtgccagtgggtctgggacagacttcaccctcaacatccatcctgtggaggaggaggatactgcaacctattactgtcagcaaagtaatgaggatccgtacacgttcggaggggggaccaagctggaaataaaa

SEQ ID NO: 84 - DNA, 332 bp, artificial
  Humanized anti-CD16A light chain variable region Hu3G8VL-1
gacatcgtgatgacccaatctccagactctttggctgtgtctctaggggagagggccaccatcaactgcaaggccagccaaagtgttgattttgatggtgatagttttatgaactggtaccaacagaaaccaggacagccacccaaactcctcatctatactacatccaatctagaatctggggtcccagacaggtttagtggcagtgggtctgggacagacttcaccctcaccatcagcagcctgcaggctgaggatgtggcagtttattactgtcagcaaagtaatgaggatccgtacacgttcggacaggggaccaagcttgagatcaa

SEQ ID NO: 85 - protein, 121 aa, artificial
  Humanized 2B6 heavy chain variable region
QVQLVQSGAEVKKPGASVKVSCKASGYTFTNYWIHWVRQAPGQGLEWIGVIDPSDTYPNYNKKFKGRVTMTVVVSTSTAYMELRSLRSDDTAVYYCARNGDSDYYSGMDYWGQGTTVTVSS

SEQ ID NO: 86 - DNA, 363 bp, artificial
  humanized 2B6 heavy chain variable region
caggttcagctggtgcagtctggagctgaggtgaagaagcctggggcctcagtgaaggtctcctgcaaggcttctggttacacctttaccaactactggatacactgggtgcgacaggcccctggacaagggcttgagtggattggagtgattgatccttctgatacttatccaaattacaataaaaagttcaagggcagagtcaccatgaccgtagtcgtatccacgagcacagcctacatggagctgaggagcctgagatctgacgacacggccgtgtattactgtgcgagaaacggtgattccgattattactctggtatggactactgggggcaagggaccacggtcaccgtctcctca

SEQ ID NO: 87 - protein, 111 aa, artificial; identical to SEQ ID NO: 71
  Humanized 2B6 light chain variable region

SEQ ID NO: 88 - DNA, 321 bp, artificial
  humanized 2B6 light chain variable region
gaaattgtgctgactcagtctccagactttcagtctgtgactccaaaggagaaagtcaccttcacctgcaggaccagtcagagcattggcacaaacatacactggtaccagcagaaaccagatcagtctccaaagctcctcatcaaggaggtttctgagtctatctctggagtcccatcgaggttcagtggcagtggatctgggacagatttcaccctcaccatcaatagcctggaagctgaagatgctgcaacgtattactgtcaacaaagtaatacctggccgttcacgttcggcggagggaccaaggtggagatcaaa

SEQ ID NO: 89 - protein, 6 aa, artificial
  thrombin cleavage recognition site
LVPRGS

SEQ ID NO: 90 - protein, 4 aa, artificial
  Factor Xa cleavage recognition site
  VARIANT (2)..(2): Xaa=Glu or Asp
IXGR

SEQ ID NO: 91 - protein, 5 aa, artificial
  enterokinase cleavage recognition site
DDDDK

SEQ ID NO: 92 - protein, 4 aa, artificial
  furin cleavage recognition site
  VARIANT (2)..(3): Xaa=any amino acid
RXXR

SEQ ID NO: 93 - protein, 4 aa, artificial
  preferred furin cleavage recognition site
  VARIANT (2)..(2): Xaa=any amino acid
  VARIANT (3)..(3): Xaa=Lys or Arg
RXXR

SEQ ID NO: 94 - protein, 7 aa, artificial
  AcTEV cleavage recognition site
QNLYFQG

SEQ ID NO: 95 - protein, 487 aa, artificial
  covalent diabody polyprotein precursor
DTVLTQSPASLAVSLGQRATISCKASQSVDFDGDSFMNWYQQKPGQPPKLLIYTTSNLESGIPARFSASGSGTDFTLNIHPVEEEDTATYYCQQSNEDPYTFGGGTKLEIKGGGSGGGGEVELVESGGGLVQPGRSLKLSCAASGFTFSDYYMAWVRQAPTTGLEWVASISYDGGDTHYRDSVKGRFTISRDNAKSSLYLQMDSLRSEDTATYYCATETTGIPTGVMDAWGQGVSVTVSSLGGCGGRAKRDVQMTQSPSNLAASPGESVSINCKASESISKYLAWYLQKPGKANKLLMYDGSTLQSGIPSRFSGSGSGTDFTLTIRSLEPEDFGLYYCQQHYEYPATFGSGTKLEIKGGGSGGGGQVTLKESGPGILQPSQTLSLTCSFSGFSLRTSGMGVGWIRQPSGKGLEWLAHIWWDDDKRYNPALKSRLTISKDTSSNQVFLKIASVDTADTATYYCAQINPAWFAYWGQGTLVTVSSLGGC

SEQ ID NO: 96 - DNA, 1464 bp, artificial
  DNA sequence of SEQ ID NO:97 (covalent diabody polyprotein precursor)
gacactgtgctgacccaatctccagcttctttggctgtgtctctagggcagagggccaccatctcctgcaaggccagccaaagtgttgattttgatggtgatagttttatgaactggtaccaacagaaaccaggacagccacccaaactcctcatctatactacatccaatctagaatctgggatcccagccaggtttagtgccagtgggtctgggacagacttcaccctcaacatccatcctgtggaggaggaggatactgcaacctattactgtcagcaaagtaatgaggatccgtacacgttcggaggggggaccaagctggaaataaaaggaggcggatccggaggcggaggcgaggtggagctagtggagtctgggggaggcttagtgcagcctggaaggtccctgaaactctcgtgtgcagcctcaggattcactttcagtgactattacatggcctgggtccggcaggctccaacgacgggtctggagtgggtcgcatccattagttatgatggtggtgacactcactatcgagactccgtgaagggccgatttactatttccagagataatgcaaaaagcagcctatacctgcaaatggacagtctgaggtctgaggacacggccacttattactgtgcaacagagactacgggaatacctacaggtgttatggatgcctggggtcaaggagtttcagtcactgtctcctcactgggaggctgcggcgggagagctaagagggatgtccagatgacccagtctccatctaatcttgctgcctctcctggagaaagtgtttccatcaattgcaaggcaagtgagagcattagcaagtatttagcctggtatctacagaaacctgggaaagcaaataagcttcttatgtacgatgggtcaactttgcaatctggaattccatcgaggttcagtggcagtggatctggtacagatttcactctcaccatcagaagcctggagcctgaagattttggactctattactgtcaacagcattatgaatatccagccacgttcggttctgggaccaagctggagatcaaaggaggcggatccggaggcggaggccaggttaccctgaaagagtctggccctgggatattgcagccctcccagaccctcagtctgacttgttctttctctgggttttcactgaggacttctggtatgggtgtaggctggattcgtcagccttcagggaagggtctagagtggctggcacacatttggtgggatgatgacaagcgctataatccagccctgaagagccgactgacaatctccaaggatacctccagcaaccaggtattcctcaaaatcgccagtgtggacactgcagatactgccacatactactgtgctcaaataaaccccgcctggtttgcttactggggccaagggactctggtcactgtgagctcactgggaggctgctag

SEQ ID NO: 97 - protein, 511 aa, artificial
  covalent diabody polyprotein precursor
DTVLTQSPASLAVSLGQRATISCKASQSVDFDGDSFMNWYQQKPGQPPKLLIYTTSNLESGIPARFSASGSGTDFTLNIHPVEEEDTATYYCQQSNEDPYTFGGGTKLEIKGGGSGGGGEVELVESGGGLVQPGRSLKLSCAASGFTFSDYYMAWVRQAPTTGLEWVASISYDGGDTHYRDSVKGRFTISRDNAKSSLYLQMDSLRSEDTATYYCATETTGIPTGVMDAWGQGVSVTVSSLGGCGGRAKRAPVKQTLNFDLLKLAGDVESNPGPDVQMTQSPSNLAASPGESVSINCKASESISKYLAWYLQKPGKANKLLMYDGSTLQSGIPSRFSGSGSGTDFTLTIRSLEPEDFGLYYCQQHYEYPATFGSGTKLEIKGGGSGGGGQVTLKESGPGILQPSQTLSLTCSFSGFSLRTSGMGVGWIRQPSGKGLEWLAHIWWDDDKRYNPALKSRLTISKDTSSNQVFLKIASVDTADTATYYCAQINPAWFAYWGQGTLVTVSSLGGC

SEQ ID NO: 98 - DNA, 1536 bp, artificial
  DNA sequence of SEQ ID NO:99 (covalent diabody polyprotein precursor)
gacactgtgctgacccaatctccagcttctttggctgtgtctctagggcagagggccaccatctcctgcaaggccagccaaagtgttgattttgatggtgatagttttatgaactggtaccaacagaaaccaggacagccacccaaactcctcatctatactacatccaatctagaatctgggatcccagccaggtttagtgccagtgggtctgggacagacttcaccctcaacatccatcctgtggaggaggaggatactgcaacctattactgtcagcaaagtaatgaggatccgtacacgttcggaggggggaccaagctggaaataaaaggaggcggatccggaggcggaggcgaggtggagctagtggagtctgggggaggcttagtgcagcctggaaggtccctgaaactctcgtgtgcagcctcaggattcactttcagtgactattacatggcctgggtccggcaggctccaacgacgggtctggagtgggtcgcatccattagttatgatggtggtgacactcactatcgagactccgtgaagggccgatttactatttccagagataatgcaaaaagcagcctatacctgcaaatggacagtctgaggtctgaggacacggccacttattactgtgcaacagagactacgggaatacctacaggtgttatggatgcctggggtcaaggagtttcagtcactgtctcctcactgggaggctgcggcgggagagctaagagggcccctgtgaagcagaccctgaacttcgacctgctgaagctggccggagacgtggagagcaaccccggccccgatgtccagatgacccagtctccatctaatcttgctgcctctcctggagaaagtgtttccatcaattgcaaggcaagtgagagcattagcaagtatttagcctggtatctacagaaacctgggaaagcaaataagcttcttatgtacgatgggtcaactttgcaatctggaattccatcgaggttcagtggcagtggatctggtacagatttcactctcaccatcagaagcctggagcctgaagattttggactctattactgtcaacagcattatgaatatccagccacgttcggttctgggaccaagctggagatcaaaggaggcggatccggaggcggaggccaggttaccctgaaagagtctggccctgggatattgcagccctcccagaccctcagtctgacttgttctttctctgggttttcactgaggacttctggtatgggtgtaggctggattcgtcagccttcagggaagggtctagagtggctggcacacatttggtgggatgatgacaagcgctataatccagccctgaagagccgactgacaatctccaaggatacctccagcaaccaggtattcctcaaaatcgccagtgtggacactgcagatactgccacatactactgtgctcaaataaaccccgcctggtttgcttactggggccaagggactctggtcactgtgagctcactgggaggctgctag

SEQ ID NO: 99 - protein, 239 aa, homo sapiens
EIVLTQSPDFQSVTPKEKVTFTCRTSQSIGTNIHWYQQKPDQSPKLLIKEVSESISGVPSRFSGSGSGTDFTLTINSLEAEDAATYYCQQSNTWPFTFGGGTKVEIKGGGSGGGGQVTLRESGPALVKPTQTLTLTCTFSGFSLSTSGMGVGWIRQPPGKALEWLAHIWWDDDKRYNPALKSRLTISKDTSKNQVVLTMTNMDPVDTATYYCAQINPAWFAYWGQGTLVTVSSFNRGEC

SEQ ID NO: 100 - DNA, 720 bp, homo sapiens
gaaattgtgctgactcagtctccagactttcagtctgtgactccaaaggagaaagtcaccttcacctgcaggaccagtcagagcattggcacaaacatacactggtaccagcagaaaccagatcagtctccaaagctcctcatcaaggaggtttctgagtctatctctggagtcccatcgaggttcagtggcagtggatctgggacagatttcaccctcaccatcaatagcctggaagctgaagatgctgcaacgtattactgtcaacaaagtaatacctggccgttcacgttcggcggagggaccaaggtggagatcaaaggaggcggatccggaggcggaggccaggttaccctgagagagtctggccctgcgctggtgaagcccacacagaccctcacactgacttgtaccttctctgggttttcactgagcacttctggtatgggtgtaggctggattcgtcagcctcccgggaaggctctagagtggctggcacacatttggtgggatgatgacaagcgctataatccagccctgaagagccgactgacaatctccaaggatacctccaaaaaccaggtagtcctcacaatgaccaacatggaccctgtggatactgccacatactactgtgctcaaataaaccccgcctggtttgcttactggggccaagggactctggtcactgtgagctcattcaacaggggagagtgttag

SEQ ID NO: 101 - protein, 246 aa, Homo sapiens
DIVMTQSPDSLAVSLGERATINCKASQSVDFDGDSFMNWYQQKPGQPPKLLIYTTSNLESGVPDRFSGSGSGTDFTLTISSLQAEDVAVYYCQQSNEDPYTFGQGTKLEIKGGGSGGGGQVQLVQSGAEVKKPGASVKVSCKASGYTFTNYWIHWVRQAPGQGLEWIGVIDPSDTYPNYNKKFKGRVTMTVVVSTSTAYMELRSLRSDDTAVYYCARNGDSDYYSGMDYWGQGTTVTVSSVEPKSC

SEQ ID NO: 102 - DNA, 741 bp, Homo sapiens
gacatcgtgatgacccaatctccagactctttggctgtgtctctaggggagagggccaccatcaactgcaaggccagccaaagtgttgattttgatggtgatagttttatgaactggtaccaacagaaaccaggacagccacccaaactcctcatctatactacatccaatctagaatctggggtcccagacaggtttagtggcagtgggtctgggacagacttcaccctcaccatcagcagcctgcaggctgaggatgtggcagtttattactgtcagcaaagtaatgaggatccgtacacgttcggacaggggaccaagcttgagatcaaaggaggcggatccggaggcggaggccaggttcagctggtgcagtctggagctgaggtgaagaagcctggggcctcagtgaaggtctcctgcaaggcttctggttacacctttaccaactactggatacactgggtgcgacaggcccctggacaagggcttgagtggattggagtgattgatccttctgatacttatccaaattacaataaaaagttcaagggcagagtcaccatgaccgtagtcgtatccacgagcacagcctacatggagctgaggagcctgagatctgacgacacggccgtgtattactgtgcgagaaacggtgattccgattattactctggtatggactactgggggcaagggaccacggtcaccgtctcctcagttgagcccaaatcttgttag

SEQ ID NO: 103 - protein, 30 aa, Artificial Sequence
  VH Sequences Derived from 3G8 VH FR1
QVTLKESGPGILQPSQTLSLTCSFSGFSLR

SEQ ID NO: 104 - protein, 30 aa, Artificial Sequence
  VH Sequences Derived from 3G8 VH FR1
QVTLRESGPALVKPTQTLTLTCTFSGFSLS

SEQ ID NO: 105 - protein, 30 aa, Artificial Sequence
  VH Sequences Derived from 3G8 VH FR1
QVTLKESGPALVKPTQTLTLTCTFSGFSLS

SEQ ID NO: 106 - protein, 30 aa, Artificial Sequence
  VH Sequences Derived from 3G8 VH FR1
QVTLRESGPALVKPTQTLTLTCTFSGFSLR

SEQ ID NO: 107 - protein, 30 aa, Artificial Sequence
  VH Sequences Derived from 3G8 VH FR1
QITLKESGPTLVKPTQTLTLTCTFSGFSLS

SEQ ID NO: 108 - protein, 7 aa, Artificial Sequence
  VH Sequences Derived from 3G8 VH *  CDR1
TSGMGVG

SEQ ID NO: 109 - protein, 7 aa, Artificial Sequence
  VH Sequences Derived from 3G8 VH *  CDR1
TSGVGVG

SEQ ID NO: 110 - protein, 14 aa, Artificial Sequence
  VH Sequences Derived from 3G8 VH * FR2
WIRQPSGKGLEWLA

SEQ ID NO: 111 - protein, 14 aa, Artificial Sequence
  VH Sequences Derived from 3G8 VH * FR2
WIRQPPGKALEWLA

SEQ ID NO: 112 - protein, 16 aa, Artificial Sequence
  VH Sequences Derived from 3G8 VH * CDR2
HIWWDDDKRYNPALKS

SEQ ID NO: 113 - protein, 16 aa, Artificial Sequence
  VH Sequences Derived from 3G8 VH * CDR2
HIYWNDDKRYNPALKS

SEQ ID NO: 114 - protein, 16 aa, Artificial Sequence
  VH Sequences Derived from 3G8 VH * CDR2
HIWWDDDKRYSPSLKS

SEQ ID NO: 115 - protein, 16 aa, Artificial Sequence
  VH Sequences Derived from 3G8 VH * CDR2
HIYWDDDKRYNPALKS

SEQ ID NO: 116 - protein, 16 aa, Artificial Sequence
  VH Sequences Derived from 3G8 VH * CDR2
HIWWNDDKRYNPALKS

SEQ ID NO: 117 - protein, 16 aa, Artificial Sequence
  VH Sequences Derived from 3G8 VH * CDR2
LIDWDDDKRYSPSLKS

SEQ ID NO: 118 - protein, 16 aa, Artificial Sequence
  VH Sequences Derived from 3G8 VH * CDR2
HIFWDDDKRYSPSLKS

SEQ ID NO: 119 - protein, 16 aa, Artificial Sequence
  VH Sequences Derived from 3G8 VH * CDR2
LIWWDDDKRYSPSLKS

SEQ ID NO: 120 - protein, 16 aa, Artificial Sequence
  VH Sequences Derived from 3G8 VH * CDR2
HIDWDDDKRYSPSLKS

SEQ ID NO: 121 - protein, 16 aa, Artificial Sequence
  VH Sequences Derived from 3G8 VH * CDR2
LIWWNDDKRYSPSLKS

SEQ ID NO: 122 - protein, 29 aa, Artificial Sequence
  VH Sequences Derived from 3G8 VH * FR3
RLTISKDTSSNQVFLKIDTADTATYYCAQ

SEQ ID NO: 123 - protein, 29 aa, Artificial Sequence
  VH Sequences Derived from 3G8 VH * FR3
RLTISKDTSKNQVVLTMDPVDTATYYCAR

SEQ ID NO: 124 - protein, 29 aa, Artificial Sequence
  VH Sequences Derived from 3G8 VH * FR3
RLTISKDTSKNQVVLTMDPVDTATYYCAQ

SEQ ID NO: 125 - protein, 29 aa, Artificial Sequence
  VH Sequences Derived from 3G8 VH * FR3
RLTISKDTSKNQVVLTMDPVDTATYYCAT

SEQ ID NO: 126 - protein, 29 aa, Artificial Sequence
  VH Sequences Derived from 3G8 VH * FR3
RLTISKDTSKNQVVLTMDPVDTATYYCAK

SEQ ID NO: 127 - protein, 29 aa, Artificial Sequence
  VH Sequences Derived from 3G8 VH * FR3
RLTISKDTSKNQVVLTMDPVDTATYYCAA

SEQ ID NO: 128 - protein, 29 aa, Artificial Sequence
  VH Sequences Derived from 3G8 VH * FR3
RLTISKDTSKNQVVLTMDPVDTATYYCAH

SEQ ID NO: 129 - protein, 29 aa, Artificial Sequence
  VH Sequences Derived from 3G8 VH * FR3
RLTITKDTSKNQVVLTMDPVDTATYYCAR

SEQ ID NO: 130 - protein, 29 aa, Artificial Sequence
  VH Sequences Derived from 3G8 VH * FR3
RLTITKDTSKNQVVLTMDPVDTATYYCAH

SEQ ID NO: 131 - protein, 29 aa, Artificial Sequence
  VH Sequences Derived from 3G8 VH * FR3
RLTITKDTSKNQVVLTMDPVDTATYYCAQ

SEQ ID NO: 132 - protein, 29 aa, Artificial Sequence
  VH Sequences Derived from 3G8 VH * FR3
RLTISKDTSSNQVFLKADTADTATYYCAQ

SEQ ID NO: 133 - protein, 29 aa, Artificial Sequence
  VH Sequences Derived from 3G8 VH * FR3
RLTISKDTSKNQVVLTTDPVDTATYYCAR

SEQ ID NO: 134 - protein, 29 aa, Artificial Sequence
  VH Sequences Derived from 3G8 VH * FR3
RLTISKDTSKNQVVLTTDPVDTATYYCAQ

SEQ ID NO: 135 - protein, 29 aa, Artificial Sequence
  VH Sequences Derived from 3G8 VH * FR3
RLTISKDTSKNQVVLTTDPVDTATYYCAT

SEQ ID NO: 136 - protein, 29 aa, Artificial Sequence
  VH Sequences Derived from 3G8 VH * FR3
RLTISKDTSKNQVVLTTDPVDTATYYCAK

SEQ ID NO: 137 - protein, 29 aa, Artificial Sequence
  VH Sequences Derived from 3G8 VH * FR3
RLTISKDTSKNQVVLTTDPVDTATYYCAA

SEQ ID NO: 138 - protein, 29 aa, Artificial Sequence
  VH Sequences Derived from 3G8 VH * FR3
RLTISKDTSKNQVVLTTDPVDTATYYCAH

SEQ ID NO: 139 - protein, 29 aa, Artificial Sequence
  VH Sequences Derived from 3G8 VH * FR3
RLTITKDTSKNQVVLTTDPVDTATYYCAR

SEQ ID NO: 140 - protein, 29 aa, Artificial Sequence
  VH Sequences Derived from 3G8 VH * FR3
RLTITKDTSKNQVVLTTDPVDTATYYCAH

SEQ ID NO: 141 - protein, 29 aa, Artificial Sequence
  VH Sequences Derived from 3G8 VH * FR3
RLTITKDTSKNQVVLTTDPVDTATYYCAQ

SEQ ID NO: 142 - protein, 29 aa, Artificial Sequence
  VH Sequences Derived from 3G8 VH * FR3
RLTISKDTSSNQVFLKSDTADTATYYCAQ

SEQ ID NO: 143 - protein, 29 aa, Artificial Sequence
  VH Sequences Derived from 3G8 VH * FR3
RLTISKDTSKNQVVLTNDPVDTATYYCAR

SEQ ID NO: 144 - protein, 29 aa, Artificial Sequence
  VH Sequences Derived from 3G8 VH * FR3
RLTISKDTSKNQVVLTNDPVDTATYYCAQ

SEQ ID NO: 145 - protein, 29 aa, Artificial Sequence
  VH Sequences Derived from 3G8 VH * FR3
RLTISKDTSKNQVVLTNDPVDTATYYCAT

SEQ ID NO: 146 - protein, 29 aa, Artificial Sequence
  VH Sequences Derived from 3G8 VH * FR3
RLTISKDTSKNQVVLTNDPVDTATYYCAK

SEQ ID NO: 147 - protein, 29 aa, Artificial Sequence
  VH Sequences Derived from 3G8 VH * FR3
RLTISKDTSKNQVVLTNDPVDTATYYCAA

SEQ ID NO: 148 - protein, 29 aa, Artificial Sequence
  VH Sequences Derived from 3G8 VH * FR3
RLTISKDTSKNQVVLTNDPVDTATYYCAH

SEQ ID NO: 149 - protein, 29 aa, Artificial Sequence
  VH Sequences Derived from 3G8 VH * FR3
RLTITKDTSKNQVVLTNDPVDTATYYCAR

SEQ ID NO: 150 - protein, 29 aa, Artificial Sequence
  VH Sequences Derived from 3G8 VH * FR3
RLTITKDTSKNQVVLTNDPVDTATYYCAH

SEQ ID NO: 151 - protein, 29 aa, Artificial Sequence
  VH Sequences Derived from 3G8 VH * FR3
RLTITKDTSKNQVVLTNDPVDTATYYCAQ

SEQ ID NO: 152 - protein, 29 aa, Artificial Sequence
  VH Sequences Derived from 3G8 VH * FR3
RLTISKDTSSNQVFLKVDTADTATYYCAQ

SEQ ID NO: 153 - protein, 29 aa, Artificial Sequence
  VH Sequences Derived from 3G8 VH * FR3
RLTISKDTSKNQVVLTMDPVDTATYYCAR

SEQ ID NO: 154 - protein, 29 aa, Artificial Sequence
  VH Sequences Derived from 3G8 VH * FR3
RLTISKDTSKNQVVLTMDPVDTATYYCAQ

SEQ ID NO: 155 - protein, 29 aa, Artificial Sequence
  VH Sequences Derived from 3G8 VH * FR3
RLTISKDTSKNQVVLTMDPVDTATYYCAT

SEQ ID NO: 156 - protein, 29 aa, Artificial Sequence
  VH Sequences Derived from 3G8 VH * FR3
RLTISKDTSKNQVVLTMDPVDTATYYCAK

SEQ ID NO: 157 - protein, 29 aa, Artificial Sequence
  VH Sequences Derived from 3G8 VH * FR3
RLTISKDTSKNQVVLTMDPVDTATYYCAA

SEQ ID NO: 158 - protein, 29 aa, Artificial Sequence
  VH Sequences Derived from 3G8 VH * FR3
RLTISKDTSKNQVVLTMDPVDTATYYCAH

SEQ ID NO: 159 - protein, 29 aa, Artificial Sequence
  VH Sequences Derived from 3G8 VH * FR3
RLTITKDTSKNQVVLTMDPVDTATYYCAR

SEQ ID NO: 160 - protein, 29 aa, Artificial Sequence
  VH Sequences Derived from 3G8 VH * FR3
RLTITKDTSKNQVVLTMDPVDTATYYCAH

SEQ ID NO: 161 - protein, 29 aa, Artificial Sequence
  VH Sequences Derived from 3G8 VH * FR3
RLTITKDTSKNQVVLTMDPVDTATYYCAQ

SEQ ID NO: 162 - protein, 8 aa, Artificial Sequence
  VH Sequences Derived from 3G8 VH * CDR3
INPAWFAY

SEQ ID NO: 163 - protein, 8 aa, Artificial Sequence
  VH Sequences Derived from 3G8 VH * CDR3
INPAWFDY

SEQ ID NO: 164 - protein, 8 aa, Artificial Sequence
  VH Sequences Derived from 3G8 VH * CDR3
INPAYFAY

SEQ ID NO: 165 - protein, 8 aa, Artificial Sequence
  VH Sequences Derived from 3G8 VH * CDR3
INPAYFDY

SEQ ID NO: 166 - protein, 11 aa, Artificial Sequence
  VH Sequences Derived from 3G8 VH * FR4
WGQGTLVTVSA

SEQ ID NO: 167 - protein, 11 aa, Artificial Sequence
  VH Sequences Derived from 3G8 VH * FR4
WGQGTLVTVSS

SEQ ID NO: 168 - protein, 15 aa, Artificial Sequence
  VL Sequences Derived from 3G8 VL* FR1
DTVLTQSPASLAVSL

SEQ ID NO: 169 - protein, 15 aa, Artificial Sequence
  VL Sequences Derived from 3G8 VL* FR1
DIVMTQSPDSLAVSL

SEQ ID NO: 170 - protein, 11 aa, Artificial Sequence
  VL Sequences Derived from 3G8 VL*  CDR1
KASQDGDSFMN

SEQ ID NO: 171 - protein, 11 aa, Artificial Sequence
  VL Sequences Derived from 3G8 VL*  CDR1
RASQDGDSFMN

SEQ ID NO: 172 - protein, 11 aa, Artificial Sequence
  VL Sequences Derived from 3G8 VL*  CDR1
KSSQDGDSFMN

SEQ ID NO: 173 - protein, 11 aa, Artificial Sequence
  VL Sequences Derived from 3G8 VL*  CDR1
KASQDGDSYMN

SEQ ID NO: 174 - protein, 11 aa, Artificial Sequence
  VL Sequences Derived from 3G8 VL*  CDR1
KASQDGDSFLN

SEQ ID NO: 175 - protein, 11 aa, Artificial Sequence
  VL Sequences Derived from 3G8 VL*  CDR1
KASQDGDSFMA

SEQ ID NO: 176 - protein, 11 aa, Artificial Sequence
  VL Sequences Derived from 3G8 VL*  CDR1
KASQDGDSYLA

SEQ ID NO: 177 - protein, 11 aa, Artificial Sequence
  VL Sequences Derived from 3G8 VL*  CDR1
KASSDGDSFMN

SEQ ID NO: 178 - protein, 11 aa, Artificial Sequence
  VL Sequences Derived from 3G8 VL*  CDR1
RASSDGDSFMN

SEQ ID NO: 179 - protein, 11 aa, Artificial Sequence
  VL Sequences Derived from 3G8 VL*  CDR1
KSSSDGDSFMN

SEQ ID NO: 180 - protein, 11 aa, Artificial Sequence
  VL Sequences Derived from 3G8 VL*  CDR1
KASSDGDSYMN

SEQ ID NO: 181 - protein, 11 aa, Artificial Sequence
  VL Sequences Derived from 3G8 VL*  CDR1
KASSDGDSFLN

SEQ ID NO: 182 - protein, 11 aa, Artificial Sequence
  VL Sequences Derived from 3G8 VL*  CDR1
KASSDGDSFMA

SEQ ID NO: 183 - protein, 11 aa, Artificial Sequence
  VL Sequences Derived from 3G8 VL*  CDR1
KASSDGDSYLA

SEQ ID NO: 184 - protein, 11 aa, Artificial Sequence
  VL Sequences Derived from 3G8 VL*  CDR1
KASVDGDSFMN

SEQ ID NO: 185 - protein, 11 aa, Artificial Sequence
  VL Sequences Derived from 3G8 VL*  CDR1
RASVDGDSFMN

SEQ ID NO: 186 - protein, 11 aa, Artificial Sequence
  VL Sequences Derived from 3G8 VL*  CDR1
KSSVDGDSFMN

SEQ ID NO: 187 - protein, 11 aa, Artificial Sequence
  VL Sequences Derived from 3G8 VL*  CDR1
KASVDGDSYMN

SEQ ID NO: 188 - protein, 11 aa, Artificial Sequence
  VL Sequences Derived from 3G8 VL*  CDR1
KASVDGDSFLN

SEQ ID NO: 189 - protein, 11 aa, Artificial Sequence
  VL Sequences Derived from 3G8 VL*  CDR1
KASVDGDSFMA

SEQ ID NO: 190 - protein, 11 aa, Artificial Sequence
  VL Sequences Derived from 3G8 VL*  CDR1
KASVDGDSYLA

SEQ ID NO: 191 - protein, 11 aa, Artificial Sequence
  VL Sequences Derived from 3G8 VL*  CDR1
KASDDGDSFMN

SEQ ID NO: 192 - protein, 11 aa, Artificial Sequence
  VL Sequences Derived from 3G8 VL*  CDR1
RASDDGDSFMN

SEQ ID NO: 193 - protein, 11 aa, Artificial Sequence
  VL Sequences Derived from 3G8 VL*  CDR1
KSSDDGDSFMN

SEQ ID NO: 194 - protein, 11 aa, Artificial Sequence
  VL Sequences Derived from 3G8 VL*  CDR1
KASDDGDSYMN

SEQ ID NO: 195 - protein, 11 aa, Artificial Sequence
  VL Sequences Derived from 3G8 VL*  CDR1
KASDDGDSFLN

SEQ ID NO: 196 - protein, 11 aa, Artificial Sequence
  VL Sequences Derived from 3G8 VL*  CDR1
KASDDGDSFMA

SEQ ID NO: 197 - protein, 11 aa, Artificial Sequence
  VL Sequences Derived from 3G8 VL*  CDR1
KASDDGDSYLA

SEQ ID NO: 198 - protein, 11 aa, Artificial Sequence
  VL Sequences Derived from 3G8 VL*  CDR1
KASFDGDSFMN

SEQ ID NO: 199 - protein, 11 aa, Artificial Sequence
  VL Sequences Derived from 3G8 VL*  CDR1
RASFDGDSFMN

SEQ ID NO: 200 - protein, 11 aa, Artificial Sequence
  VL Sequences Derived from 3G8 VL*  CDR1
KSSFDGDSFMN

SEQ ID NO: 201 - protein, 11 aa, Artificial Sequence
  VL Sequences Derived from 3G8 VL*  CDR1
KASFDGDSYMN

SEQ ID NO: 202 - protein, 11 aa, Artificial Sequence
  VL Sequences Derived from 3G8 VL*  CDR1
KASFDGDSFLN

SEQ ID NO: 203 - protein, 11 aa, Artificial Sequence
  VL Sequences Derived from 3G8 VL*  CDR1
KASFDGDSFMA

SEQ ID NO: 204 - protein, 11 aa, Artificial Sequence
  VL Sequences Derived from 3G8 VL*  CDR1
KASFDGDSYLA

SEQ ID NO: 205 - protein, 16 aa, Artificial Sequence
  VL Sequences Derived from 3G8 VL*  FR2
WYQQKAPGQPPKLLIY

SEQ ID NO: 206 - protein, 7 aa, Artificial Sequence
  VL Sequences Derived from 3G8 VL*  CDR2
TTSNLES

SEQ ID NO: 207 - protein, 7 aa, Artificial Sequence
  VL Sequences Derived from 3G8 VL*  CDR2
DASNLES

SEQ ID NO: 208 - protein, 7 aa, Artificial Sequence
  VL Sequences Derived from 3G8 VL*  CDR2
WASNLES

SEQ ID NO: 209 - protein, 7 aa, Artificial Sequence
  VL Sequences Derived from 3G8 VL*  CDR2
TTSNLET

SEQ ID NO: 210 - protein, 7 aa, Artificial Sequence
  VL Sequences Derived from 3G8 VL*  CDR2
DASNLET

SEQ ID NO: 211 - protein, 7 aa, Artificial Sequence
  VL Sequences Derived from 3G8 VL*  CDR2
DASNLAT

SEQ ID NO: 212 - protein, 7 aa, Artificial Sequence
  VL Sequences Derived from 3G8 VL*  CDR2
SASNLQS

SEQ ID NO: 213 - protein, 7 aa, Artificial Sequence
  VL Sequences Derived from 3G8 VL*  CDR2
STSNLES

SEQ ID NO: 214 - protein, 7 aa, Artificial Sequence
  VL Sequences Derived from 3G8 VL*  CDR2
STSNLQS

SEQ ID NO: 215 - protein, 7 aa, Artificial Sequence
  VL Sequences Derived from 3G8 VL*  CDR2
TTSNLQS

SEQ ID NO: 216 - protein, 7 aa, Artificial Sequence
  VL Sequences Derived from 3G8 VL*  CDR2
TTSSLQS

SEQ ID NO: 217 - protein, 32 aa, Artificial Sequence
  VL Sequences Derived from 3G8 VL*  FR3
GIPARFSASGSGTDFTLNIHPVEEEDTATYYC

SEQ ID NO: 218 - protein, 32 aa, Artificial Sequence
  VL Sequences Derived from 3G8 VL*  FR3
GVPDRFSGSGSGTDFTLTISSLQAEDVAVYYC

SEQ ID NO: 219 - protein, 9 aa, Artificial Sequence
  VL Sequences Derived from 3G8 VL*  CDR3
QQSNEDPYT

SEQ ID NO: 220 - protein, 9 aa, Artificial Sequence
  VL Sequences Derived from 3G8 VL*  CDR3
QQSYSTPYT

SEQ ID NO: 221 - protein, 9 aa, Artificial Sequence
  VL Sequences Derived from 3G8 VL*  CDR3
QQSYEDPYT

SEQ ID NO: 222 - protein, 9 aa, Artificial Sequence
  VL Sequences Derived from 3G8 VL*  CDR3
QQSNSDPYT

SEQ ID NO: 223 - protein, 9 aa, Artificial Sequence
  VL Sequences Derived from 3G8 VL*  CDR3
QQSNETPYT

SEQ ID NO: 224 - protein, 10 aa, Artificial Sequence
  VL Sequences Derived from 3G8 VL*  FR4
FGGGTKLEIK

SEQ ID NO: 225 - protein, 10 aa, Artificial Sequence
  VL Sequences Derived from 3G8 VL*  FR4
FGQGTKLEIK

SEQ ID NO: 226 - DNA, 714 bp, Artificial Sequence
  H3G8VL-CB3.1VH
gacatcgtgatgacccaatctccagactctttggctgtgtctctaggggagagggccaccatcaactgcaaggccagccaaagtgttgattttgatggtgatagttttatgaactggtaccaacagaaaccaggacagccacccaaactcctcatctatactacatccaatctagaatctggggtcccagacaggtttagtggcagtgggtctgggacagacttcaccctcaccatcagcagcctgcaggctgaggatgtggcagtttattactgtcagcaaagtaatgaggatccgtacacgttcggacaggggaccaagcttgagatcaaaggaggcggatccggaggcggaggccaggtccaactgcagcagcctggggctgagctggtgaggcctggggcttcagtgaagctgtcctgcaaggcttctggctacaccttcaccagctactggatgaactgggtgaagcagaggcctggacaaggccttgaatggattggtatggttgatccttcagacagtgaaactcactacaatcaaatgttcaaggacaaggccacattgactgttgacaaatcctccagcacagcctacatgcagctcagcagcctgacatctgaggactctgcggtctattactgtgcaagagctatgggctactggggtcaaggaacctcagtcaccgtctcctcagttgagcccaaatcttgt

SEQ ID NO: 227 - protein, 238 aa, Artificial Sequence
  H3G8VL-CB3.1VH
DIVMTQSPDSLAVSLGERATINCKASQSVDFDGDSFMNWYQQKPGQPPKLLIYTTSNLESGVPDRFSGSGSGTDFTLTISSLQAEDVAVYYCQQSNEDPYTFGQGTKLEIKGGGSGGGGQVQLQQPGAELVRPGASVKLSCKASGYTFTSYWMNWVKQRPGQGLEWIGMVDPSDSETHYNQMFKDKATLTVDKSSSTAYMQLSSLTSEDSAVYYCARAMGYWGQGTSVTVSSVEPKSC

SEQ ID NO: 228 - DNA, 732 bp, Artificial Sequence
  CB3.1VL-h3G8VH
gatgttgtgatgacccagactccactcactttgtcggttaacattggacaaccagcctccatctcttgtaagtcaagtcagagcctcttagatactgatggaaagacatatttgaattggttgttacagaggccaggccagtctccaaaccgcctaatctatctggtgtctaaactggactctggagtccctgacaggttcactggcagtggatcagggacagatttcacactgaaaatcagcagagtggaggctgaggatttgggaatttattattgctggcaaggtacacattttccgctcacgttcggtgctgggaccaagctggagctgaaaggaggcggatccggaggcggaggccaggttaccctgagagagtctggccctgcgctggtgaagcccacacagaccctcacactgacttgtaccttctctgggttttcactgagcacttctggtatgggtgtaggctggattcgtcagcctcccgggaaggctctagagtggctggcacacatttggtgggatgatgacaagcgctataatccagccctgaagagccgactgacaatctccaaggatacctccaaaaaccaggtagtcctcacaatgaccaacatggaccctgtggatactgccacatactactgtgctcaaataaaccccgcctggtttgcttactggggccaagggactctggtcactgtgagctcattcaacaggggagagtgt

SEQ ID NO: 229 - protein, 244 aa, Artificial Sequence
  CB3.1VL-h3G8VH
DVVMTQTPLTLSVNIGQPASISCKSSQSLLDTDGKTYLNWLLQRPGQSPNRLIYLVSKLDSGVPDRFTGSGSGTDFTLKISRVEAEDLGIYYCWQGTHFPLTFGAGTKLELKGGGSGGGGQVTLRESGPALVKPTQTLTLTCTFSGFSLSTSGMGVGWIRQPPGKALEWLAHIWWDDDKRYNPALKSRLTISKDTSKNQVVLTMTNMDPVDTATYYCAQINPAWFAYWGQGTLVTVSSFNRGEC

SEQ ID NO: 230 - DNA, 702 bp, Artificial Sequence
  8B5-CB3.1-VEPKSC
gacattcagatgacacagtctccatcctccctacttgcggcgctgggagaaagagtcagtctcacttgtcgggcaagtcaggaaattagtggttacttaagctggcttcagcagaaaccagatggaactattaaacgcctgatctacgccgcatccactttagattctggtgtcccaaaaaggttcagtggcagtgagtctgggtcagattattctctcaccatcagcagtcttgagtctgaagattttgcagactattactgtctacaatattttagttatccgctcacgttcggtgctgggaccaagctggagctgaaaggaggcggatccggaggcggaggccaggtccaactgcagcagcctggggctgagctggtgaggcctggggcttcagtgaagctgtcctgcaaggcttctggctacaccttcaccagctactggatgaactgggtgaagcagaggcctggacaaggccttgaatggattggtatggttgatccttcagacagtgaaactcactacaatcaaatgttcaaggacaaggccacattgactgttgacaaatcctccagcacagcctacatgcagctcagcagcctgacatctgaggactctgcggtctattactgtgcaagagctatgggctactggggtcaaggaacctcagtcaccgtctcctcagttgagcccaaatcttgt

SEQ ID NO: 231 - protein, 234 aa, Artificial Sequence
  8B5-CB3.1-VEPKSC
DIQMTQSPSSLLAALGERVSLTCRASQEISGYLSWLQQKPDGTIKRLIYAASTLDSGVPKRFSGSESGSDYSLTISSLESEDFADYYCLQYFSYPLTFGAGTKLELKGGGSGGGGQVQLQQPGAELVRPGASVKLSCKASGYTFTSYWMNWVKQRPGQGLEWIGMVDPSDSETHYNQMFKDKATLTVDKSSSTAYMQLSSLTSEDSAVYYCARAMGYWGQGTSVTVSSVEPKSC

SEQ ID NO: 232 - DNA, 726 bp, Artificial Sequence
  CB3.1-8B5-FNRGEC
gatgttgtgatgacccagactccactcactttgtcggttaacattggacaaccagcctccatctcttgtaagtcaagtcagagcctcttagatactgatggaaagacatatttgaattggttgttacagaggccaggccagtctccaaaccgcctaatctatctggtgtctaaactggactctggagtccctgacaggttcactggcagtggatcagggacagatttcacactgaaaatcagcagagtggaggctgaggatttgggaatttattattgctggcaaggtacacattttccgctcacgttcggtgctgggaccaagctggagctgaaaggaggcggatccggaggcggaggcgaagtgaagcttgaggagtctggaggaggcttggtgcaacctggaggatccatgaaactctcttgtgaagcctctggattcacttttagtgacgcctggatggactgggtccgtcagtctccagagaaggggcttgagtgggttgctgaaattagaaacaaagctaaaaatcatgcaacatactatgctgagtctgtgatagggaggttcaccatctcaagagatgattccaaaagtagtgtctacctgcaaatgaacagcttaagagctgaagacactggcatttattactgtggggctctgggccttgactactggggccaaggcaccactctcacagtctcctcgttcaacaggggagagtgt

SEQ ID NO: 233 - protein, 242 aa, Artificial Sequence
  CB3.1-8B5-FNRGEC
DVVMTQTPLTLSVNIGQPASISCKSSQSLLDTDGKTYLNWLLQRPGQSPNRLIYLVSKLDSGVPDRFTGSGSGTDFTLKISRVEAEDLGIYYCWQGTHFPLTFGAGTKLELKGGGSGGGGEVKLEESGGGLVQPGGSMKLSCEASGFTFSDAWMDWVRQSPEKGLEWVAEIRNKAKNHATYYAESVIGRFTISRDDSKSSVYLQMNSLRAEDTGIYYCGALGLDYWGQGTTLTVSSFNRGEC

SEQ ID NO: 234 - DNA, 696 bp, Artificial Sequence
  8B5VL-CB3.1VH-LGGC
gacattcagatgacacagtctccatcctccctacttgcggcgctgggagaaagagtcagtctcacttgtcgggcaagtcaggaaattagtggttacttaagctggcttcagcagaaaccagatggaactattaaacgcctgatctacgccgcatccactttagattctggtgtcccaaaaaggttcagtggcagtgagtctgggtcagattattctctcaccatcagcagtcttgagtctgaagattttgcagactattactgtctacaatattttagttatccgctcacgttcggtgctgggaccaagctggagctgaaaggaggcggatccggaggcggaggccaggtccaactgcagcagcctggggctgagctggtgaggcctggggcttcagtgaagctgtcctgcaaggcttctggctacaccttcaccagctactggatgaactgggtgaagcagaggcctggacaaggccttgaatggattggtatggttgatccttcagacagtgaaactcactacaatcaaatgttcaaggacaaggccacattgactgttgacaaatcctccagcacagcctacatgcagctcagcagcctgacatctgaggactctgcggtctattactgtgcaagagctatgggctactggggtcaaggaacctcagtcaccgtctcctcactgggaggctgc

SEQ ID NO: 235 - protein, 232 aa, Artificial Sequence
  8B5VL-CB3.1VH-LGGC
DIQMTQSPSSLLAALGERVSLTCRASQEISGYLSWLQQKPDGTIKRLIYAASTLDSGVPKRFSGSESGSDYSLTISSLESEDFADYYCLQYFSYPLTFGAGTKLELKGGGSGGGGQVQLQQPGAELVRPGASVKLSCKASGYTFTSYWMNWVKQRPGQGLEWIGMVDPSDSETHYNQMFKDKATLTVDKSSSTAYMQLSSLTSEDSAVYYCARAMGYWGQGTSVTVSSLGGC

SEQ ID NO: 236 - DNA, 720 bp, Artificial Sequence
  CB3.1-8B5-LGGC
gatgttgtgatgacccagactccactcactttgtcggttaacattggacaaccagcctccatctcttgtaagtcaagtcagagcctcttagatactgatggaaagacatatttgaattggttgttacagaggccaggccagtctccaaaccgcctaatctatctggtgtctaaactggactctggagtccctgacaggttcactggcagtggatcagggacagatttcacactgaaaatcagcagagtggaggctgaggatttgggaatttattattgctggcaaggtacacattttccgctcacgttcggtgctgggaccaagctggagctgaaaggaggcggatccggaggcggaggcgaagtgaagcttgaggagtctggaggaggcttggtgcaacctggaggatccatgaaactctcttgtgaagcctctggattcacttttagtgacgcctggatggactgggtccgtcagtctccagagaaggggcttgagtgggttgctgaaattagaaacaaagctaaaaatcatgcaacatactatgctgagtctgtgatagggaggttcaccatctcaagagatgattccaaaagtagtgtctacctgcaaatgaacagcttaagagctgaagacactggcatttattactgtggggctctgggccttgactactggggccaaggcaccactctcacagtctcctcgctgggaggctgc

SEQ ID NO: 237 - protein, 240 aa, Artificial Sequence
  CB3.1-8B5-LGGC
DVVMTQTPLTLSVNIGQPASISCKSSQSLLDTDGKTYLNWLLQRPGQSPNRLIYLVSKLDSGVPDRFTGSGSGTDFTLKISRVEAEDLGIYYCWQGTHFPLTFGAGTKLELKGGGSGGGGEVKLEESGGGLVQPGGSMKLSCEASGFTFSDAWMDWVRQSPEKGLEWVAEIRNKAKNHATYYAESVIGRFTISRDDSKSSVYLQMNSLRAEDTGIYYCGALGLDYWGQGTTLTVSSLGGC

SEQ ID NO: 238 - DNA, 47 bp, Artificial Sequence
  Lgh628F Primer
ggaggcggatccggaggcggaggccaggtccaactgcagcagcctgg

SEQ ID NO: 239 - DNA, 49 bp, Artificial Sequence
  Lgh629R Primer
tttgaattctaacaagatttgggctcaactgaggagacggtgactgagg

SEQ ID NO: 240 - DNA, 45 bp, Artificial Sequence
  Lgh630R Primer
gcctccgcctccggatccgcctcctttcagctccagcttggtccc

SEQ ID NO: 241 - DNA, 47 bp, Artificial Sequence
  Lgh631F Primer
ggaggcggatccggaggcggaggcgaagtgaagcttgaggagtctgg

SEQ ID NO: 242 - DNA, 49 bp, Artificial Sequence
  Lgh640R Primer
tttgaattctaacactctcccctgttgaacgaggagactgtgagagtgg

SEQ ID NO: 243 - DNA, 48 bp, Artificial Sequence
  Lgh644R Primer
tttgtcgtcatcatcgtctttgtagtcggagtggacacctgtggagag

SEQ ID NO: 244 - DNA, 42 bp, Artificial Sequence
  Lgh646R Primer
tttgaattctagcagcctcccagtgaggagacggtgactgag

SEQ ID NO: 245 - DNA, 45 bp, Artificial Sequence
  Lgh647F Primer
caaagacgatgatgacgacaaagacattcagatgacacagtctcc

SEQ ID NO: 246 - DNA, 43 bp, Artificial Sequence
  Lgh648R Primer
tttgaattctagcagcctcccagcgaggagactgtgagagtgg

SEQ ID NO: 247 - DNA, 1044 bp, Artificial Sequence
  2.4G2-3G8-hKappa
gatgtccagatgacccagtctccatctaatcttgctgcctctcctggagaaagtgtttccatcaattgcaaggcaagtgagagcattagcaagtatttagcctggtatctacagaaacctgggaaagcaaataagcttcttatgtacgatgggtcaactttgcaatctggaattccatcgaggttcagtggcagtggatctggtacagatttcactctcaccatcagaagcctggagcctgaagattttggactctattactgtcaacagcattatgaatatccagccacgttcggttctgggaccaagctggagatcaaaggaggcggatccggaggcggaggccaggttaccctgaaagagtctggccctgggatattgcagccctcccagaccctcagtctgacttgttctttctctgggttttcactgaggacttctggtatgggtgtaggctggattcgtcagccttcagggaagggtctagagtggctggcacacatttggtgggatgatgacaagcgctataatccagccctgaagagccgactgacaatctccaaggatacctccagcaaccaggtattcctcaaaatcgccagtgtggacactgcagatactgccacatactactgtgctcaaataaaccccgcctggtttgcttactggggccaagggactctggtcactgtgagctcactgggaggctgcggcggagggagccgtacggtggctgcaccatcggtcttcatcttcccgccatctgatgagcagttgaaatctggaactgcctctgttgtgtgcctgctgaataacttctatcccagagaggccaaagtacagtggaaggtggataacgccctccaatcgggtaactcccaggagagtgtcacagagcaggacagcaaggacagcacctacagcctcagcagcaccctgacgctgagcaaagcagactacgagaaacacaaagtctacgcctgcgaagtcacccatcagggcctgagctcgcccgtcacaaagagcttcaacaggggagagtgt

SEQ ID NO: 248 - protein, 348 aa, Artificial Sequence
  2.4G2-3G8-hKappa
DVQMTQSPSNLAASPGESVSINCKASESISKYLAWYLQKPGKANKLLMYDGSTLQSGIPSRFSGSGSGTDFTLTIRSLEPEDFGLYYCQQHYEYPATFGSGTKLEIKGGGSGGGGQVTLKESGPGILQPSQTLSLTCSFSGFSLRTSGMGVGWIRQPSGKGLEWLAHIWWDDDKRYNPALKSRLTISKDTSSNQVFLKIASVDTADTATYYCAQINPAWFAYWGQGTLVTVSSLGGCGGGSRTVAAPSVFIFPPSDEQLKSGTASVVCLLNNFYPREAKVQWKVDNALQSGNSQESVTEQDSKDSTYSLSSTLTLSKADYEKHKVYACEVTHQGLSSPVTKSFNRGEC

SEQ ID NO: 249 - DNA, 1734 bp, Artificial Sequence
  3G8-2.4G2-hG1
gacactgtgctgacccaatctccagcttctttggctgtgtctctagggcagagggccaccatctcctgcaaggccagccaaagtgttgattttgatggtgatagttttatgaactggtaccaacagaaaccaggacagccacccaaactcctcatctatactacatccaatctagaatctgggatcccagccaggtttagtgccagtgggtctgggacagacttcaccctcaacatccatcctgtggaggaggaggatactgcaacctattactgtcagcaaagtaatgaggatccgtacacgttcggaggggggaccaagctggaaataaaaggaggcggatccggaggcggaggcgaggtggagctagtggagtctgggggaggcttagtgcagcctggaaggtccctgaaactctcgtgtgcagcctcaggattcactttcagtgactattacatggcctgggtccggcaggctccaacgacgggtctggagtgggtcgcatccattagttatgatggtggtgacactcactatcgagactccgtgaagggccgatttactatttccagagataatgcaaaaagcagcctatacctgcaaatggacagtctgaggtctgaggacacggccacttattactgtgcaacagagactacgggaatacctacaggtgttatggatgcctggggtcaaggagtttcagtcactgtctcctcactgggaggctgcggcggagggagcgcctccaccaagggcccatcggtcttccccctggcaccctcctccaagagcacctctgggggcacagcggccctgggctgcctggtcaaggactacttccccgaaccggtgacggtgtcgtggaactcaggcgccctgaccagcggcgtgcacaccttcccggctgtcctacagtcctcaggactctactccctcagcagcgtggtgaccgtgccctccagcagcttgggcacccagacctacatctgcaacgtgaatcacaagcccagcaacaccaaggtggacaagagagttgagcccaaatcttgtgacaaaactcacacatgcccaccgtgcccagcacctgaactcctggggggaccgtcagtcttcctcttccccccaaaacccaaggacaccctcatgatctcccggacccctgaggtcacatgcgtggtggtggacgtgagccacgaagaccctgaggtcaagttcaactggtacgtggacggcgtggaggtgcataatgccaagacaaagccgcgggaggagcagtacaacagcacgtaccgtgtggtcagcgtcctcaccgtcctgcaccaggactggctgaatggcaaggagtacaagtgcaaggtctccaacaaagccctcccagcccccatcgagaaaaccatctccaaagccaaagggcagccccgagaaccacaggtgtacaccctgcccccatcccgggatgagctgaccaagaaccaggtcagcctgacctgcctggtcaaaggcttctatcccagcgacatcgccgtggagtgggagagcaatgggcagccggagaacaactacaagaccacgcctcccgtgctggactccgacggctccttcttcctctacagcaagctcaccgtggacaagagcaggtggcagcaggggaacgtcttctcatgctccgtgatgcatgaggctctgcacaaccactacacgcagaagagcctctccctgtctccgggtaaa

SEQ ID NO: 250 - protein, 578 aa, Artificial Sequence
  3G8-2.4G2-hG1
DTVLTQSPASLAVSLGQRATISCKASQSVDFDGDSFMNWYQQKPGQPPKLLIYTTSNLESGIPARFSASGSGTDFTLNIHPVEEEDTATYYCQQSNEDPYTFGGGTKLEIKGGGSGGGGEVELVESGGGLVQPGRSLKLSCAASGFTFSDYYMAWVRQAPTTGLEWVASISYDGGDTHYRDSVKGRFTISRDNAKSSLYLQMDSLRSEDTATYYCATETTGIPTGVMDAWGQGVSVTVSSLGGCGGGSASTKGPSVFPLAPSSKSTSGGTAALGCLVKDYFPEPVTVSWNSGALTSGVHTFPAVLQSSGLYSLSSVVTVPSSSLGTQTYICNVNHKPSNTKVDKRVEPKSCDKTHTCPPCPAPELLGGPSVFLFPPKPKDTLMISRTPEVTCVVVDVSHEDPEVKFNWYVDGVEVHNAKTKPREEQYNSTYRVVSVLTVLHQDWLNGKEYKCKVSNKALPAPIEKTISKAKGQPREPQVYTLPPSRDELTKNQVSLTCLVKGFYPSDIAVEWESNGQPENNYKTTPPVLDSDGSFFLYSKLTVDKSRWQQGNVFSCSVMHEALHNHYTQKSLSLSPGK

SEQ ID NO: 251 - DNA, 720 bp, Artificial Sequence
  CD79VL-CD32BVH
gatgttgtgatgactcagtctccactctccctgcccgtcacccttggacagccggcctccatctcctgcaagtcaagtcagagcctcttagatagtgatggaaagacatatttgaattggtttcagcagaggccaggccaatctccaaaccgcctaatttatctggtgtctaaactggactctggggtcccagacagattcagcggcagtgggtcaggcactgatttcacactgaaaatcagcagggtggaggctgaggatgttggggtttattactgctggcaaggtacacattttccgctcacgttcggcggagggaccaagcttgagatcaaaggaggcggatccggaggcggaggcgaagtgaagcttgaggagtctggaggaggcttggtgcaacctggaggatccatgaaactctcttgtgaagcctctggattcacttttagtgacgcctggatggactgggtccgtcagtctccagagaaggggcttgagtgggttgctgaaattagaaacaaagctaaaaatcatgcaacatactatgctgagtctgtgatagggaggttcaccatctcaagagatgattccaaaagtagtgtctacctgcaaatgaacagcttaagagctgaagacactggcatttattactgtggggctctgggccttgactactggggccaaggcaccactctcacagtctcctcgctgggaggctgc

SEQ ID NO: 252 - protein, 240 aa, Artificial Sequence
  CD79VL-CD32BVH
DVVMTQSPLSLPVTLGQPASISCKSSQSLLDSDGKTYLNWFQQRPGQSPNRLIYLVSKLDSGVPDRFSGSGSGTDFTLKISRVEAEDVGVYYCWQGTHFPLTFGGGTKLEIKGGGSGGGGEVQLVESGGGLVQPGGSLRLSCAASGFTFSDAWMDWVRQAPGKGLEWVAEIRNKAKNHATYYAESVIGRFTISRDDAKNSLYLQMNSLRAEDTAVYYCGALGLDYWGQGTLVTVSSLGGC

SEQ ID NO: 253 - DNA, 696 bp, Artificial Sequence
  CD32BVL-CD79VH-1
gacatccagatgacccagtctccatcctccttatctgcctctgtgggagatagagtcaccatcacttgtcgggcaagtcaggaaattagtggttacttaagctggctgcagcagaaaccaggcaaggcccctagacgcctgatctacgccgcatccactttagattctggtgtcccatccaggttcagtggcagtgagtctgggaccgagttcaccctcaccatcagcagccttcagcctgaagattttgcaacctattactgtctacaatattttagttatccgctcacgttcggaggggggaccaaggtggaaataaaaggaggcggatccggaggcggaggccaggttcagctggtgcagtctggagctgaggtgaagaagcctggcgcctcagtgaaggtctcctgcaaggcttctggttacacctttaccagctactggatgaactgggtgcgacaggcccctggacaagggcttgagtggatcggaatgattgatccttcagacagtgaaactcactacaatcaaatgttcaaggacagagtcaccatgaccacagacacatccacgagcacagcctacatggagctgaggagcctgagatctgacgacacggccgtgtattactgtgcgagagctatgggctactgggggcaagggaccacggtcaccgtctcctcactgggaggctgc

SEQ ID NO: 254 - protein, 232 aa, Artificial Sequence
  CD32BVL-CD79VH-1
DIQMTQSPSSLSASVGDRVTITCRASQEISGYLSWLQQKPGKAPRRLIYAASTLDSGVPSRFSGSESGTEFTLTISSLQPEDFATYYCLQYFSYPLTFGGGTKVEIKGGGSGGGGQVQLVQSGAEVKKPGASVKVSCKASGYTFTSYWMNWVRQAPGQGLEWIGMIDPSDSETHYNQMFKDRVTMTTDTSTSTAYMELRSLRSDDTAVYYCARAMGYWGQGTTVTVSSLGGC

SEQ ID NO: 255 - DNA, 696 bp, Artificial Sequence
  CD32BVL-CD79VH-2
gacatccagatgacccagtctccatcctccttatctgcctctgtgggagatagagtcaccatcacttgtcgggcaagtcaggaaattagtggttacttaagctggctgcagcagaaaccaggcaaggcccctagacgcctgatctacgccgcatccactttagattctggtgtcccatccaggttcagtggcagtgagtctgggaccgagttcaccctcaccatcagcagccttcagcctgaagattttgcaacctattactgtctacaatattttagttatccgctcacgttcggaggggggaccaaggtggaaataaaaggaggcggatccggaggcggaggccaggttcagctggtgcagtctggagctgaggtgaagaagcctggcgcctcagtgaaggtctcctgcaaggcttctggttacacctttaccagctactggatgaactgggtgcgacaggcccctggacaagggcttgagtggatcggaatgattgatccttcagacagtgaaactcactacaatcaaaagttcaaggacagagtcaccatgaccacagacacatccacgagcacagcctacatggagctgaggagcctgagatctgacgacacggccgtgtattactgtgcgagagctatgggctactgggggcaagggaccacggtcaccgtctcctcactgggaggctgc

SEQ ID NO: 256 - protein, 232 aa, Artificial Sequence
  CD32BVL-CD79VH-2
DIQMTQSPSSLSASVGDRVTITCRASQEISGYLSWLQQKPGKAPRRLIYAASTLDSGVPSRFSGSESGTEFTLTISSLQPEDFATYYCLQYFSYPLTFGGGTKVEIKGGGSGGGGQVQLVQSGAEVKKPGASVKVSCKASGYTFTSYWMNWVRQAPGQGLEWIGMIDPSDSETHYNQKFKDRVTMTTDTSTSTAYMELRSLRSDDTAVYYCARAMGYWGQGTTVTVSSLGGC

SEQ ID NO: 257 - DNA, 720 bp, Artificial Sequence; identical to SEQ ID NO: 251
  hHBCRCVL. R45N-h8B5VH-LGGC

SEQ ID NO: 258 - protein, 240 aa, Artificial Sequence; identical to SEQ ID NO: 252
  hHBCRCVL. R45N-h8B5VH-LGGC

SEQ ID NO: 259 - DNA, 696 bp, Artificial Sequence; identical to SEQ ID NO: 253
  H8B5VL-hHBCRCVH M48I-LGGC

SEQ ID NO: 260 - protein, 232 aa, Artificial Sequence; identical to SEQ ID NO: 254
  H8B5VL-HBCRCVH M48I-LGGC

SEQ ID NO: 261 - DNA, 36 bp, Artificial Sequence; identical to SEQ ID NO: 55
  Lgh321F Primer

SEQ ID NO: 262 - DNA, 45 bp, Artificial Sequence
  Lgh386R Primer
tttgaattctagcagcctcccagtgaggagacggtgaccgtggtc

SEQ ID NO: 263 - DNA, 39 bp, Artificial Sequence
  Lgh784F Primer
ggcggatccggaggcggaggccaggttcagctggtgcag

SEQ ID NO: 264 - DNA, 38 bp, Artificial Sequence
  Lgh785R Primer
cctccggatccgcctcctttgatctcaagcttggtccc

SEQ ID NO: 265 - DNA, 42 bp, Artificial Sequence
  Lgh786R Primer
tttgaattctagcagcctcccaggctggagacggtcaccagg

SEQ ID NO: 266 - DNA, 44 bp, Artificial Sequence
  Lgh787F Primer
ggaggcggatccggaggcggaggcgaagtgcagcttgtggagtc

SEQ ID NO: 267 - protein, 8 aa, Artificial Sequence
  Linker
LGGCGGGS

SEQ ID NO: 268 - protein, 4 aa, Artificial Sequence
  Linker
LEIK

SEQ ID NO: 269 - protein, 4 aa, Artificial Sequence
  Linker
TVSS

SEQ ID NO: 270 - protein, 343 aa, Artificial Sequence
  H8B5VL-hBCRCVH M48I, M62K_LGGCG3S_hKappa
DIQMTQSPSSLSASVGDRVTITCRASQEISGYLSWLQQKPGKAPRRLIYAASTLDSGVPSRFSGSESGTEFTLTISSLQPEDFATYYCLQYFSYPLTFGGGTKVEIKGGGSGGGGQVQLVQSGAEVKKPGASVKVSCKASGYTFTSYWMNWVRQAPGQGLEWIGMIDPSDSETHYNQKFKDRVTMTTDTSTSTAYMELRSLRSDDTAVYYCARAMGYWGQGTTVTVSSLGGCGGGSRTVAAPSVFIFPPSDEQLKSGTASVVCLLNNFYPREAKVQWKVDNALQSGNSQESVTEQDSKDSTYSLSSTLTLSKADYEKHKVYACEVTHQGLSSPVTKSFNRGEC

SEQ ID NO: 271 - DNA, 1032 bp, Artificial Sequence
  H8B5VL-hBCRCVH M48I, M62K_LGGCG3S_hKappa
gacatccagatgacccagtctccatcctccttatctgcctctgtgggagatagagtcaccatcacttgtcgggcaagtcaggaaattagtggttacttaagctggctgcagcagaaaccaggcaaggcccctagacgcctgatctacgccgcatccactttagattctggtgtcccatccaggttcagtggcagtgagtctgggaccgagttcaccctcaccatcagcagccttcagcctgaagattttgcaacctattactgtctacaatattttagttatccgctcacgttcggaggggggaccaaggtggaaataaaaggaggcggatccggaggcggaggccaggttcagctggtgcagtctggagctgaggtgaagaagcctggcgcctcagtgaaggtctcctgcaaggcttctggttacacctttaccagctactggatgaactgggtgcgacaggcccctggacaagggcttgagtggatcggaatgattgatccttcagacagtgaaactcactacaatcaaaagttcaaggacagagtcaccatgaccacagacacatccacgagcacagcctacatggagctgaggagcctgagatctgacgacacggccgtgtattactgtgcgagagctatgggctactgggggcaagggaccacggtcaccgtctcctcactgggaggctgcggcggagggagccgaactgtggctgcaccatcggtcttcatcttcccgccatctgatgagcagttgaaatctggaactgcctctgttgtgtgcctgctgaataacttctatcccagagaggccaaagtacagtggaaggtggataacgccctccaatcgggtaactcccaggagagtgtcacagagcaggacagcaaggacagcacctacagcctcagcagcaccctgacgctgagcaaagcagactacgagaaacacaaagtctacgcctgcgaagtcacccatcagggcctgagctcgcccgtcacaaagagcttcaacaggggagagtgttag

SEQ ID NO: 272 - protein, 574 aa, Artificial Sequence
  HBCRCVL R45N-h8B5VH_LGGCGGGS-hG1
DVVMTQSPLSLPVTLGQPASISCKSSQSLLDSDGKTYLNWFQQRPGQSPNRLIYLVSKLDSGVPDRFSGSGSGTDFTLKISRVEAEDVGVYYCWQGTHFPLTFGGGTKLEIKGGGSGGGGEVQLVESGGGLVQPGGSLRLSCAASGFTFSDAWMDWVRQAPGKGLEWVAEIRNKAKNHATYYAESVIGRFTISRDDAKNSLYLQMNSLRAEDTAVYYCGALGLDYWGQGTLVTVSSLGGCGGGSASTKGPSVFPLAPSSKSTSGGTAALGCLVKDYFPEPVTVSWNSGALTSGVHTFPAVLQSSGLYSLSSVVTVPSSSLGTQTYICNVNHKPSNTKVDKRVEPKSCDKTHTCPPCPAPELLGGPSVFLFPPKPKDTLMISRTPEVTCVVVDVSHEDPEVKFNWYVDGVEVHNAKTKPREEQYNSTYRVVSVLTVLHQDWLNGKEYKCKVSNKALPAPIEKTISKAKGQPREPQVYTLPPSRDELTKNQVSLTCLVKGFYPSDIAVEWESNGQPENNYKTTPPVLDSDGSFFLYSKLTVDKSRWQQGNVFSCSVMHEALHNHYTQKSLSLSPGK

SEQ ID NO: 273 - DNA, 1722 bp, Artificial Sequence
  HBCRCVL R45N-h8B5VH_LGGCGGGS-hG1
gatgttgtgatgactcagtctccactctccctgcccgtcacccttggacagccggcctccatctcctgcaagtcaagtcagagcctcttagatagtgatggaaagacatatttgaattggtttcagcagaggccaggccaatctccaaaccgcctaatttatctggtgtctaaactggactctggggtcccagacagattcagcggcagtgggtcaggcactgatttcacactgaaaatcagcagggtggaggctgaggatgttggggtttattactgctggcaaggtacacattttccgctcacgttcggcggagggaccaagcttgagatcaaaggaggcggatccggaggcggaggcgaagtgcagcttgtggagtctggaggaggcttggtgcaacctggaggatccctgagactctcttgtgccgcctctggattcacttttagtgacgcctggatggactgggtccgtcaggccccaggcaaggggcttgagtgggttgctgaaattagaaacaaagctaaaaatcatgcaacatactatgctgagtctgtgatagggaggttcaccatctcaagagatgacgccaaaaacagtctgtacctgcaaatgaacagcttaagagctgaagacactgccgtgtattactgtggggctctgggccttgactactggggccaaggcaccctggtgaccgtctccagcctgggaggctgcggcggagggagcgcctccaccaagggcccatcggtcttccccctggcaccctcctccaagagcacctctgggggcacagcggccctgggctgcctggtcaaggactacttccccgaaccggtgacggtgtcgtggaactcaggcgccctgaccagcggcgtgcacaccttcccggctgtcctacagtcctcaggactctactccctcagcagcgtggtgaccgtgccctccagcagcttgggcacccagacctacatctgcaacgtgaatcacaagcccagcaacaccaaggtggacaagagagttgagcccaaatcttgtgacaaaactcacacatgcccaccgtgcccagcacctgaactcctggggggaccgtcagtcttcctcttccccccaaaacccaaggacaccctcatgatctcccggacccctgaggtcacatgcgtggtggtggacgtgagccacgaagaccctgaggtcaagttcaactggtacgtggacggcgtggaggtgcataatgccaagacaaagccgcgggaggagcagtacaacagcacgtaccgtgtggtcagcgtcctcaccgtcctgcaccaggactggctgaatggcaaggagtacaagtgcaaggtctccaacaaagccctcccagcccccatcgagaaaaccatctccaaagccaaagggcagccccgagaaccacaggtgtacaccctgcccccatcccgggatgagctgaccaagaaccaggtcagcctgacctgcctggtcaaaggcttctatcccagcgacatcgccgtggagtgggagagcaatgggcagccggagaacaactacaagaccacgcctcccgtgctggactccgacggctccttcttcctctacagcaagctcaccgtggacaagagcaggtggcagcaggggaacgtcttctcatgctccgtgatgcatgaggctctgcacaaccactacacgcagaagagcctctccctgtctccgggtaaa

SEQ ID NO: 274 - protein, 335 aa, Artificial Sequence
  H8B5VL-HBCRCVH M48I, M62K_(-4)LEIK_hKappa
DIQMTQSPSSLSASVGDRVTITCRASQEISGYLSWLQQKPGKAPRRLIYAASTLDSGVPSRFSGSESGTEFTLTISSLQPEDFATYYCLQYFSYPLTFGGGTKVEIKGGGSGGGGQVQLVQSGAEVKKPGASVKVSCKASGYTFTSYWMNWVRQAPGQGLEWIGMIDPSDSETHYNQKFKDRVTMTTDTSTSTAYMELRSLRSDDTAVYYCARAMGYWGQGTTVLEIKRTVAAPSVFIFPPSDEQLKSGTASVVCLLNNFYPREAKVQWKVDNALQSGNSQESVTEQDSKDSTYSLSSTLTLSKADYEKHKVYACEVTHQGLSSPVTKSFNRGEC

SEQ ID NO: 275 - DNA, 1005 bp, Artificial Sequence
  H8B5VL-HBCRCVH M48I, M62K_(-4)LEIK_hKappa
gacatccagatgacccagtctccatcctccttatctgcctctgtgggagatagagtcaccatcacttgtcgggcaagtcaggaaattagtggttacttaagctggctgcagcagaaaccaggcaaggcccctagacgcctgatctacgccgcatccactttagattctggtgtcccatccaggttcagtggcagtgagtctgggaccgagttcaccctcaccatcagcagccttcagcctgaagattttgcaacctattactgtctacaatattttagttatccgctcacgttcggaggggggaccaaggtggaaataaaaggaggcggatccggaggcggaggccaggttcagctggtgcagtctggagctgaggtgaagaagcctggcgcctcagtgaaggtctcctgcaaggcttctggttacacctttaccagctactggatgaactgggtgcgacaggcccctggacaagggcttgagtggatcggaatgattgatccttcagacagtgaaactcactacaatcaaaagttcaaggacagagtcaccatgaccacagacacatccacgagcacagcctacatggagctgaggagcctgagatctgacgacacggccgtgtattactgtgcgagagctatgggctactgggggcaagggaccacggtcctggagatcaagcgaactgtggctgcaccatcggtcttcatcttcccgccatctgatgagcagttgaaatctggaactgcctctgttgtgtgcctgctgaataacttctatcccagagaggccaaagtacagtggaaggtggataacgccctccaatcgggtaactcccaggagagtgtcacagagcaggacagcaaggacagcacctacagcctcagcagcaccctgacgctgagcaaagcagactacgagaaacacaaagtctacgcctgcgaagtcacccatcagggcctgagctcgcccgtcacaaagagcttcaacaggggagagtgt

SEQ ID NO: 276 - protein, 566 aa, Artificial Sequence
  HBCRCVL R45N-h8B5VH_(-4)TVSS-hG1  = HBCRCVL R45N-h8B5VH_-hG1
DVVMTQSPLSLPVTLGQPASISCKSSQSLLDSDGKTYLNWFQQRPGQSPNRLIYLVSKLDSGVPDRFSGSGSGTDFTLKISRVEAEDVGVYYCWQGTHFPLTFGGGTKLEIKGGGSGGGGEVQLVESGGGLVQPGGSLRLSCAASGFTFSDAWMDWVRQAPGKGLEWVAEIRNKAKNHATYYAESVIGRFTISRDDAKNSLYLQMNSLRAEDTAVYYCGALGLDYWGQGTLVTVSSASTKGPSVFPLAPSSKSTSGGTAALGCLVKDYFPEPVTVSWNSGALTSGVHTFPAVLQSSGLYSLSSVVTVPSSSLGTQTYICNVNHKPSNTKVDKRVEPKSCDKTHTCPPCPAPELLGGPSVFLFPPKPKDTLMISRTPEVTCVVVDVSHEDPEVKFNWYVDGVEVHNAKTKPREEQYNSTYRVVSVLTVLHQDWLNGKEYKCKVSNKALPAPIEKTISKAKGQPREPQVYTLPPSRDELTKNQVSLTCLVKGFYPSDIAVEWESNGQPENNYKTTPPVLDSDGSFFLYSKLTVDKSRWQQGNVFSCSVMHEALHNHYTQKSLSLSPGK

SEQ ID NO: 277 - DNA, 1698 bp, Artificial Sequence
  HBCRCVL R45N-h8B5VH_(-4)TVSS-hG1
gatgttgtgatgactcagtctccactctccctgcccgtcacccttggacagccggcctccatctcctgcaagtcaagtcagagcctcttagatagtgatggaaagacatatttgaattggtttcagcagaggccaggccaatctccaaaccgcctaatttatctggtgtctaaactggactctggggtcccagacagattcagcggcagtgggtcaggcactgatttcacactgaaaatcagcagggtggaggctgaggatgttggggtttattactgctggcaaggtacacattttccgctcacgttcggcggagggaccaagcttgagatcaaaggaggcggatccggaggcggaggcgaagtgcagcttgtggagtctggaggaggcttggtgcaacctggaggatccctgagactctcttgtgccgcctctggattcacttttagtgacgcctggatggactgggtccgtcaggccccaggcaaggggcttgagtgggttgctgaaattagaaacaaagctaaaaatcatgcaacatactatgctgagtctgtgatagggaggttcaccatctcaagagatgacgccaaaaacagtctgtacctgcaaatgaacagcttaagagctgaagacactgccgtgtattactgtggggctctgggccttgactactggggccaaggcaccctggtgaccgtctccagcgcctccaccaagggcccatcggtcttccccctggcaccctcctccaagagcacctctgggggcacagcggccctgggctgcctggtcaaggactacttccccgaaccggtgacggtgtcgtggaactcaggcgccctgaccagcggcgtgcacaccttcccggctgtcctacagtcctcaggactctactccctcagcagcgtggtgaccgtgccctccagcagcttgggcacccagacctacatctgcaacgtgaatcacaagcccagcaacaccaaggtggacaagagagttgagcccaaatcttgtgacaaaactcacacatgcccaccgtgcccagcacctgaactcctggggggaccgtcagtcttcctcttccccccaaaacccaaggacaccctcatgatctcccggacccctgaggtcacatgcgtggtggtggacgtgagccacgaagaccctgaggtcaagttcaactggtacgtggacggcgtggaggtgcataatgccaagacaaagccgcgggaggagcagtacaacagcacgtaccgtgtggtcagcgtcctcaccgtcctgcaccaggactggctgaatggcaaggagtacaagtgcaaggtctccaacaaagccctcccagcccccatcgagaaaaccatctccaaagccaaagggcagccccgagaaccacaggtgtacaccctgcccccatcccgggatgagctgaccaagaaccaggtcagcctgacctgcctggtcaaaggcttctatcccagcgacatcgccgtggagtgggagagcaatgggcagccggagaacaactacaagaccacgcctcccgtgctggactccgacggctccttcttcctctacagcaagctcaccgtggacaagagcaggtggcagcaggggaacgtcttctcatgctccgtgatgcatgaggctctgcacaaccactacacgcagaagagcctctccctgtctccgggtaaa

SEQ ID NO: 278 - protein, 10 aa, Artificial Sequence
  Linker
FNRGECGGGS

SEQ ID NO: 279 - protein, 13 aa, Artificial Sequence
  Linker
FNRGECLQVYYRM

SEQ ID NO: 280 - protein, 6 aa, Artificial Sequence
  Linker
LEGEEG

SEQ ID NO: 281 - protein, 7 aa, Artificial Sequence
  Linker
LEGEEGC

SEQ ID NO: 282 - protein, 4 aa, Artificial Sequence
  Linker
LEIK

SEQ ID NO: 283 - protein, 5 aa, Artificial Sequence
  Linker
LGEEG

SEQ ID NO: 284 - protein, 6 aa, Artificial Sequence
  Linker
LGEEGC

SEQ ID NO: 285 - protein, 8 aa, Artificial Sequence
  Linker
LGGCGGGS

SEQ ID NO: 286 - protein, 5 aa, Artificial Sequence
  Linker
LGKKG

SEQ ID NO: 287 - protein, 6 aa, Artificial Sequence
  Linker
LGKKGC

SEQ ID NO: 288 - protein, 6 aa, Artificial Sequence
  Linker
LKGKKG

SEQ ID NO: 289 - protein, 7 aa, Artificial Sequence
  Linker
LKGKKGC

SEQ ID NO: 290 - protein, 7 aa, Artificial Sequence
  Linker
LQVYYRM

SEQ ID NO: 291 - protein, 8 aa, Artificial Sequence
  Linker
LQVYYRMC

SEQ ID NO: 292 - protein, 4 aa, Artificial Sequence
  Linker
TVSS

SEQ ID NO: 293 - protein, 10 aa, Artificial Sequence
  Linker
VEPKSCGGGS

SEQ ID NO: 294 - protein, 14 aa, Artificial Sequence
  Linker
VEPKSCYLYLRARV

SEQ ID NO: 295 - protein, 7 aa, Artificial Sequence
  Linker
VQVHYRM

SEQ ID NO: 296 - protein, 8 aa, Artificial Sequence
  Linker
VQVHYRMC

SEQ ID NO: 297 - protein, 8 aa, Artificial Sequence
  Linker
YLYLRARV

SEQ ID NO: 298 - protein, 9 aa, Artificial Sequence
  Linker
YLYLRARVC

SEQ ID NO: 299 - protein, 28 aa, Artificial Sequence
  E-coil Linker
EVAALEKEVAALEKEVAALEKEVAALEK

SEQ ID NO: 300 - protein, 28 aa, Artificial Sequence
  K-coil Linker
KVAALKEKVAALKEKVAALKEKVAALKE

SEQ ID NO: 301 - protein, 5 aa, Artificial Sequence
  Linker
GGGNS

SEQ ID NO: 302 - protein, 107 aa, Artificial Sequence; identical to SEQ ID NO: 41
  YA2B6 light chain variable region

SEQ ID NO: 303 - protein, 121 aa, Artificial Sequence; identical to SEQ ID NO: 38
  YA2B6 hheavy chain variable region

SEQ ID NO: 304 - protein, 46 aa, Artificial Sequence
  Albumin Binding Domain
LAEAKVLANRELDKYGVSDYYKNLINNAKTVEGVKALIDEILAALP

SEQ ID NO: 305 - protein, 279 aa, Artificial Sequence
  h3G8VL1-G3SG4-h2B6VH4-Kcoil-GGGNS
DIVMTQSPDSLAVSLGERATINCKASQSVDFDGDSFMNWYQQKPGQPPKLLIYTTSNLESGVPDRFSGSGSGTDFTLTISSLQAEDVAVYYCQQSNEDPYTFGQGTKLEIKGGGSGGGGQVQLVQSGAEVKKPGASVKVSCKASGYTFTNYWIHWVRQAPGQGLEWIGVIDPSDTYPNYNKKFKGRVTMTVVVSTSTAYMELRSLRSDDTAVYYCARNGDSDYYSGMDYWGQGTTVTVSSGGCGGGKVAALKEKVAALKEKVAALKEKVAALKEGGGNS

SEQ ID NO: 306 - DNA, 837 bp, Artificial Sequence
  h3G8VL1-G3SG4-h2B6VH4-Kcoil-GGGNS
gacatcgtgatgacccaatctccagactctttggctgtgtctctaggggagagggccaccatcaactgcaaggccagccaaagtgttgattttgatggtgatagttttatgaactggtaccaacagaaaccaggacagccacccaaactcctcatctatactacatccaatctagaatctggggtcccagacaggtttagtggcagtgggtctgggacagacttcaccctcaccatcagcagcctgcaggctgaggatgtggcagtttattactgtcagcaaagtaatgaagatccgtacacgttcggacaggggaccaagcttgagatcaaaggaggcggatccggcggcggaggccaggttcagctggtgcagtctggagctgaggtgaagaagcctggggcctcagtgaaggtctcctgcaaggcttctggttacacctttaccaactactggatacactgggtgcgacaggcccctggacaagggcttgagtggattggagtgattgatccttctgatacttatccaaattacaataaaaagttcaagggcagagtcaccatgaccgtagtcgtatccacgagcacagcctacatggagctgaggagcctgagatctgacgacacggccgtgtattactgtgcgagaaacggtgattccgattattactctggtatggactactgggggcaagggaccacggtcaccgtctcctccggaggatgtggcggtggaaaagtggccgcactgaaggagaaagttgctgctttgaaagagaaggtcgccgcacttaaggaaaaggtcgcagccctgaaagagggcggcgggaattct

SEQ ID NO: 307 - protein, 318 aa, Artificial Sequence
  h2B6VL5-G3SG4-h3G8VH5-Ecoil-GGGNS-ABD
EIVLTQSPDFQSVTPKEKVTFTCRTSQSIGTNIHWYQQKPDQSPKLLIKEVSESISGVPSRFSGSGSGTDFTLTINSLEAEDAATYYCQQSNTWPFTFGGGTKVEIKGGGSGGGGQVTLRESGPALVKPTQTLTLTCTFSGFSLSTSGMGVGWIRQPPGKALEWLAHIWWDDDKRYNPALKSRLTISKDTSKNQVVLTMTNMDPVDTATYYCAQINPAWFAYWGQGTLVTVSSGGCGGGEVAALEKEVAALEKEVAALEKEVAALEKGGGNSLAEAKVLANRELDKYGVSDYYKNLINNAKTVEGVKALIDEILAALP

SEQ ID NO: 308 - DNA, 954 bp, Artificial Sequence
  h2B6VL5-G3SG4-h3G8VH5-Ecoil-GGGNS-ABD
gaaattgtgctgactcagtctccagactttcagtctgtgactccaaaggagaaagtcaccttcacctgcaggaccagtcagagcattggcacaaacatacactggtaccagcagaaaccagatcagtctccaaagctcctcatcaaggaggtttctgagtctatctctggagtcccatcgaggttcagtggcagtggatctgggacagatttcaccctcaccatcaatagcctggaagctgaagatgctgcaacgtattactgtcaacaaagtaatacctggccgttcacgttcggcggagggaccaaggtggagatcaaaggaggcggatccggcggcggaggccaggttaccctgagagagtctggccctgcgctggtgaagcccacacagaccctcacactgacttgtaccttctctgggttttcactgagcacttctggtatgggtgtaggctggattcgtcagcctcccgggaaggctctagagtggctggcacacatttggtgggatgatgacaagcgctataatccagccctgaagagccgactgacaatctccaaggatacctccaaaaaccaggtagtcctcacaatgaccaacatggaccctgtggatactgccacatactactgtgctcaaataaaccccgcctggtttgcttactggggccaagggactctggtcactgtgagctccggaggatgtggcggtggagaagtggccgcactggagaaagaggttgctgctttggagaaggaggtcgctgcacttgaaaaggaggtcgcagccctggagaaaggcggcgggaattctctggccgaagcaaaagtgctggccaaccgcgaactggataaatatggcgtgagcgattattataagaacctgattaacaacgcaaagaccgtggaaggcgtgaaagcactgattgatgaaattctggccgccctgcct

SEQ ID NO: 309 - protein, 5 aa, Artificial Sequence
  Linker
APSSS

SEQ ID NO: 310 - protein, 8 aa, Artificial Sequence
  Linker
VPSMGSSS

SEQ ID NO: 311 - protein, 383 aa, Homo sapiens
MGLGPVFLLLAGIFPFAPPGAAAEPHSLRYNLTVLSWDGSVQSGFLTEVHLDGQPFLRCDRQKCRAKPQGQWAEDVLGNKTWDRETRDLTGNGKDLRMTLAHIKDQKEGLHSLQEIRVCEIHEDNSTRSSQHFYYDGELFLSQNLETKEWTMPQSSRAQTLAMNVRNFLKEDAMKTKTHYHAMHADCLQELRRYLKSGVVLRRTVPPMVNVTRSEASEGNITVTCRASGFYPWNITLSWRQDGVSLSHDTQQWGDVLPDGNGTYQTWVATRICQGEEQRFTCYMEHSGNHSTHPVPSGKVLVLQSHWQTFHVSAVAAAAIFVIIIFYVRCCKKKTSAAEGPELVSLQVLDQHPVGTSDHRDATQLGFQPLMSDLGSTGSTEGA

SEQ ID NO: 312 - protein, 305 aa, Homo sapiens
PHSLRYNLMVLSQDGSVQSGFLAEGHLDGQPFLRYDRQKRRAKPQGQWAEDVLGAKTWDTETEDLTENGQDLRRTLTHIKDQKGGLHSLQEIRVCEIHEDSSTRGSRHFYYDGELFLSQNLETQESTVPQSSRAQTLAMNVTNFWKEDAMKTKTHYRAMQADCLQKLQLPPMVNVICSEVSEGNITVTCRASSFYPRNITLTWRQDGVSLSHNTQQWGDVLPDGNGTYQTWVATRIRQGEEQRFTCYMEHSGNHGTHPVPSGKALVLQSQRTDFPYVSAAMPCFVIIIILCVPCCKKKTSAAEGP

SEQ ID NO: 313 - protein, 7 aa, Artificial Sequence
  Linker
GFNRGEC

SEQ ID NO: 314 - protein, 7 aa, Artificial Sequence
  Linker
GVEPKSC

SEQ ID NO: 315 - protein, 241 aa, Artificial Sequence
  TCRVL-HER2VH
EIVLTQSPATLSLSPGERATLSCSATSSVSYMHWYQQKPGKAPKRWIYDTSKLASGVPSRFSGSGSGTEFTLTISSLQPEDFATYYCQQWSSNPLTFGQGTKLEIKGGGSGGGGQVQLQQSGPELVKPGASLKLSCTASGFNIKDTYIHWVKQRPEQGLEWIGRIYPTNGYTRYDPKFQDKATITADTSSNTAYLQVSRLTSEDTAVYYCSRWGGDGFYAMDYWGQGASVTVSSGFNRGEC

SEQ ID NO: 316 - DNA, 723 bp, Artificial Sequence
  TCRVL-HER2VH
gaaattgtgttgacacagtctccagccaccctgtctttgtctccaggggaaagagccaccctctcctgcagtgccacctcaagtgtaagttacatgcactggtatcagcagaaaccagggaaagcccctaagcgctggatctatgacacatccaaactggcttctggggtcccatcaaggttcagcggcagtggatctgggacagaatttactctcacaatcagcagcctgcagcctgaagattttgcaacttattactgtcagcagtggagtagtaacccgctcacgtttggccaggggaccaagcttgagatcaaaggaggcggatccggcggcggaggccaggttcagctgcagcagtctgggccagagcttgtgaagccaggggcctcactcaagttgtcctgtacagcttctggcttcaacattaaagacacctatatacactgggtgaaacagaggcctgaacagggcctggaatggattggaaggatttatcctacgaatggttatactagatatgacccgaagttccaggacaaggccactataacagcagacacatcctccaacacagcctacctgcaggtcagccgcctgacatctgaggacactgccgtctattattgttctagatggggaggggacggcttctatgctatggactactggggtcaaggagcctcggtcaccgtgagctccggattcaacaggggagagtgt

SEQ ID NO: 317 - protein, 242 aa, Artificial Sequence
  HER2VL-TCRVH
DIVMTQSHKFMSTSVGDRVSITCKASQDVNTAVAWYQQKPGHSPKLLIYSASFRYTGVPDRFTGSRSGTDFTFTISSVQAEDLAVYYCQQHYTTPPTFGGGTKVEIKGGGSGGGGQVQLVQSGAEVKKPGASVKVSCKASGYKFTSYVMHWVRQAPGQGLEWIGYINPYNDVTKYNEKFKGRVTITADKSTSTAYMELSSLRSEDTAVHYCARGSYYDYDGFVYWGQGTLVTVSSGVEPKSC

SEQ ID NO: 318 - DNA, 726 bp, Artificial Sequence
  HER2VL-TCRVH
gacatcgtgatgacccagtcccacaagttcatgtccacctctgtgggcgatagggtcagcatcacctgcaaggccagccaggatgtgaatactgctgtagcctggtatcagcagaaaccaggacattctcccaaactgctgatttactccgcatccttccggtacactggagtccctgatcgcttcactggcagcagatctgggacagatttcactttcaccatcagcagtgtgcaggctgaagacctggcagtttattactgtcagcaacattatactacacctcccaccttcggagggggtaccaaggtggagatcaaaggaggcggatccggcggcggaggccaggttcagctggtgcagtctggagctgaggtgaagaagcctggggcctcagtgaaggtctcctgcaaggccagcggttacaagtttaccagctacgtgatgcactgggtgcgacaggcccctggacaagggcttgagtggatcggatatattaatccttacaatgatgttactaagtacaatgagaagttcaaaggcagagtcacgattaccgcggacaaatccacgagcacagcctacatggagctgagcagcctgagatccgaggacacggccgtgcactactgtgcgagagggagctactatgattacgacgggtttgtttactggggccaagggactctggtcactgtgagctccggagttgagcccaaatcttgt

SEQ ID NO: 319 - protein, 273 aa, Artificial Sequence
  TCRVL-HER2VH-E coil
EIVLTQSPATLSLSPGERATLSCSATSSVSYMHWYQQKPGKAPKRWIYDTSKLASGVPSRFSGSGSGTEFTLTISSLQPEDFATYYCQQWSSNPLTFGQGTKLEIKGGGSGGGGQVQLQQSGPELVKPGASLKLSCTASGFNIKDTYIHWVKQRPEQGLEWIGRIYPTNGYTRYDPKFQDKATITADTSSNTAYLQVSRLTSEDTAVYYCSRWGGDGFYAMDYWGQGASVTVSSGGCGGGEVAALEKEVAALEKEVAALEKEVAALEKGGGNS

SEQ ID NO: 320 - protein, 819 aa, Artificial Sequence
  TCRVL-HER2VH-E coil
GAAATTGTGTTGACACAGTCTCCAGCCACCCTGTCTTTGTCTCCAGGGGAAAGAGCCACCCTCTCCTGCAGTGCCACCTCAAGTGTAAGTTACATGCACTGGTATCAGCAGAAACCAGGGAAAGCCCCTAAGCGCTGGATCTATGACACATCCAAACTGGCTTCTGGGGTCCCATCAAGGTTCAGCGGCAGTGGATCTGGGACAGAATTTACTCTCACAATCAGCAGCCTGCAGCCTGAAGATTTTGCAACTTATTACTGTCAGCAGTGGAGTAGTAACCCGCTCACGTTTGGCCAGGGGACCAAGCTTGAGATCAAAGGAGGCGGATCCGGCGGCGGAGGCCAGGTTCAGCTGCAGCAGTCTGGGCCAGAGCTTGTGAAGCCAGGGGCCTCACTCAAGTTGTCCTGTACAGCTTCTGGCTTCAACATTAAAGACACCTATATACACTGGGTGAAACAGAGGCCTGAACAGGGCCTGGAATGGATTGGAAGGATTTATCCTACGAATGGTTATACTAGATATGACCCGAAGTTCCAGGACAAGGCCACTATAACAGCAGACACATCCTCCAACACAGCCTACCTGCAGGTCAGCCGCCTGACATCTGAGGACACTGCCGTCTATTATTGTTCTAGATGGGGAGGGGACGGCTTCTATGCTATGGACTACTGGGGTCAAGGAGCCTCGGTCACCGTGAGCTCCGGAGGATGTGGCGGTGGAGAAGTGGCCGCACTGGAGAAAGAGGTTGCTGCTTTGGAGAAGGAGGTCGCTGCACTTGAAAAGGAGGTCGCAGCCCTGGAGAAAGGCGGCGGGAATTCT

SEQ ID NO: 321 - protein, 274 aa, Artificial Sequence
  HER2VL-TCRVH-K coil
DIVMTQSHKFMSTSVGDRVSITCKASQDVNTAVAWYQQKPGHSPKLLIYSASFRYTGVPDRFTGSRSGTDFTFTISSVQAEDLAVYYCQQHYTTPPTFGGGTKVEIKGGGSGGGGQVQLVQSGAEVKKPGASVKVSCKASGYKFTSYVMHWVRQAPGQGLEWIGYINPYNDVTKYNEKFKGRVTITADKSTSTAYMELSSLRSEDTAVHYCARGSYYDYDGFVYWGQGTLVTVSSGGCGGGKVAALKEKVAALKEKVAALKEKVAALKEGGGNS

SEQ ID NO: 322 - DNA, 822 bp, Artificial Sequence
  HER2VL-TCRVH-K coil
gacatcgtgatgacccagtcccacaagttcatgtccacctctgtgggcgatagggtcagcatcacctgcaaggccagccaggatgtgaatactgctgtagcctggtatcagcagaaaccaggacattctcccaaactgctgatttactccgcatccttccggtacactggagtccctgatcgcttcactggcagcagatctgggacagatttcactttcaccatcagcagtgtgcaggctgaagacctggcagtttattactgtcagcaacattatactacacctcccaccttcggagggggtaccaaggtggagatcaaaggaggcggatccggcggcggaggccaggttcagctggtgcagtctggagctgaggtgaagaagcctggggcctcagtgaaggtctcctgcaaggccagcggttacaagtttaccagctacgtgatgcactgggtgcgacaggcccctggacaagggcttgagtggatcggatatattaatccttacaatgatgttactaagtacaatgagaagttcaaaggcagagtcacgattaccgcggacaaatccacgagcacagcctacatggagctgagcagcctgagatccgaggacacggccgtgcactactgtgcgagagggagctactatgattacgacgggtttgtttactggggccaagggactctggtcactgtgagctccggaggatgtggcggtggaaaagtggccgcactgaaggagaaagttgctgctttgaaagagaaggtcgccgcacttaaggaaaaggtcgcagccctgaaagagggcggcgggaattct